European Patent Application EP 4 644 419 A1, published November 5, 2025. Title: Antibody targeting CD112R or antigen-binding fragment thereof and use thereof. Applicant: HANGZHOU ZHONGMEIHUADONG PHARMACEUTICAL CO., LTD. The sequence listing filed with the application follows.

SEQUENCE LISTING (662 sequences)

SEQ ID NO: 1 - protein, 5 aa, Synthetic construct
DYYLN

SEQ ID NO: 2 - protein, 5 aa, Synthetic construct
DYYIN

SEQ ID NO: 3 - protein, 5 aa, Synthetic construct
DYFMN

SEQ ID NO: 4 - protein, 5 aa, Synthetic construct
AYYIN

SEQ ID NO: 5 - protein, 5 aa, Synthetic construct
DYYMN

SEQ ID NO: 6 - protein, 5 aa, Synthetic construct
DYYMF

SEQ ID NO: 7 - protein, 5 aa, Synthetic construct
DIYMH

SEQ ID NO: 8 - protein, 5 aa, Synthetic construct
DSYMC

SEQ ID NO: 9 - protein, 5 aa, Synthetic construct
DYYMY

SEQ ID NO: 10 - protein, 5 aa, Synthetic construct
SYWMH

SEQ ID NO: 11 - protein, 5 aa, Synthetic construct
DYNIH

SEQ ID NO: 12 - protein, 5 aa, Synthetic construct
GYGIN

SEQ ID NO: 13 - protein, 5 aa, Synthetic construct
DYYIA

SEQ ID NO: 14 - protein, 5 aa, Synthetic construct
TYGMS

SEQ ID NO: 15 - protein, 5 aa, Synthetic construct
GYWIE

SEQ ID NO: 16 - protein, 5 aa, Synthetic construct
SYNIH

SEQ ID NO: 17 - protein, 5 aa, Synthetic construct
TYWMH

SEQ ID NO: 18 - protein, 5 aa, Synthetic construct
DSYIN

SEQ ID NO: 19 - protein, 5 aa, Synthetic construct
SYWMQ

SEQ ID NO: 20 - protein, 5 aa, Synthetic construct
DYEMH

SEQ ID NO: 21 - protein, 5 aa, Synthetic construct
DYYMS

SEQ ID NO: 22 - protein, 5 aa, Synthetic construct
GYALS

SEQ ID NO: 23 - protein, 5 aa, Synthetic construct
DYALS

SEQ ID NO: 24 - protein, 5 aa, Synthetic construct
DYYMH

SEQ ID NO: 25 - protein, 6 aa, Synthetic construct
SNYYWN

SEQ ID NO: 26 - protein, 5 aa, Synthetic construct
SYSMS

SEQ ID NO: 27 - protein, 5 aa, Synthetic construct
SYIMS

SEQ ID NO: 28 - protein, 5 aa, Synthetic construct
SYFMS

SEQ ID NO: 29 - protein, 5 aa, Synthetic construct
SYWIT

SEQ ID NO: 30 - protein, 5 aa, Synthetic construct
HYYKN

SEQ ID NO: 31 - protein, 5 aa, Synthetic construct
HYYVN

SEQ ID NO: 32 - protein, 5 aa, Synthetic construct
NYGMS

SEQ ID NO: 33 - protein, 5 aa, Synthetic construct
GYYVN

SEQ ID NO: 34 - protein, 5 aa, Synthetic construct
DYFIS

SEQ ID NO: 35 - protein, 5 aa, Synthetic construct
DYSMN

SEQ ID NO: 36 - protein, 5 aa, Synthetic construct
ASAMH

SEQ ID NO: 37 - protein, 5 aa, Synthetic construct
DYGMY

SEQ ID NO: 38 - protein, 5 aa, Synthetic construct
GYYIN

SEQ ID NO: 39 - protein, 5 aa, Synthetic construct
DYGMH

SEQ ID NO: 40 - protein, 5 aa, Synthetic construct
DYNVD

SEQ ID NO: 41 - protein, 5 aa, Synthetic construct
NYGIS

SEQ ID NO: 42 - protein, 5 aa, Synthetic construct
DYNMD

SEQ ID NO: 43 - protein, 5 aa, Synthetic construct
DYSMD

SEQ ID NO: 44 - protein, 5 aa, Synthetic construct
DYNID

SEQ ID NO: 45 - protein, 5 aa, Synthetic construct
DTYIH

SEQ ID NO: 46 - protein, 5 aa, Synthetic construct
SHGIS

SEQ ID NO: 47 - protein, 5 aa, Synthetic construct
SSWMH

SEQ ID NO: 48 - protein, 5 aa, Synthetic construct
DYNLD

SEQ ID NO: 49 - protein, 5 aa, Synthetic construct
NSWIN

SEQ ID NO: 50 - protein, 5 aa, Synthetic construct
SYTMS

SEQ ID NO: 51 - protein, 5 aa, Synthetic construct
DYWMQ

SEQ ID NO: 52 - protein, 5 aa, Synthetic construct
TYIMS

SEQ ID NO: 53 - protein, 5 aa, Synthetic construct
DYFIN

SEQ ID NO: 54 - protein, 5 aa, Synthetic construct
NFAMS

SEQ ID NO: 55 - protein, 5 aa, Synthetic construct
SFAMS

SEQ ID NO: 56 - protein, 5 aa, Synthetic construct
DYWIE

SEQ ID NO: 57 - protein, 5 aa, Synthetic construct
DYWIN

SEQ ID NO: 58 - protein, 5 aa, Synthetic construct
ENYMY

SEQ ID NO: 59 - protein, 5 aa, Synthetic construct
SYAMS

SEQ ID NO: 60 - protein, 5 aa, Synthetic construct
NYWMN

SEQ ID NO: 61 - protein, 5 aa, Synthetic construct
DFFIN

SEQ ID NO: 62 - protein, 7 aa, Synthetic construct
TFGLGIG

SEQ ID NO: 63 - protein, 5 aa, Synthetic construct
DYWIQ

SEQ ID NO: 64 - protein, 17 aa, Synthetic construct
WIFPGSESTFYNEKFKG

SEQ ID NO: 65 - protein, 17 aa, Synthetic construct
WIFPGSDYTYYNEKFKG

SEQ ID NO: 66 - protein, 17 aa, Synthetic construct
DIIPNNDSPNYNQKFKG

SEQ ID NO: 67 - protein, 17 aa, Synthetic construct
WIFPGSDSTYYNEKFKG

SEQ ID NO: 68 - protein, 17 aa, Synthetic construct
DINPNNGGTNFNQKFKG

SEQ ID NO: 69 - protein, 17 aa, Synthetic construct
TISDGGGYIYYPDSVKG

SEQ ID NO: 70 - protein, 17 aa, Synthetic construct
RIDPTNGNSEYDPRFRG

SEQ ID NO: 71 - protein, 17 aa, Synthetic construct
TISDGGGLTYYPDSVKG

SEQ ID NO: 72 - protein, 17 aa, Synthetic construct
DIHPNNGSPNYNQKFKG

SEQ ID NO: 73 - protein, 17 aa, Synthetic construct
TISDGGGYTYYPDSVKG

SEQ ID NO: 74 - protein, 17 aa, Synthetic construct
DINPNNGSPNYNQKFKG

SEQ ID NO: 75 - protein, 17 aa, Synthetic construct
VIDASDSNTKYNQKFKG

SEQ ID NO: 76 - protein, 17 aa, Synthetic construct
TISDGGGFIYYPDSVKG

SEQ ID NO: 77 - protein, 17 aa, Synthetic construct
TISDAGGYTYYPDSVKG

SEQ ID NO: 78 - protein, 17 aa, Synthetic construct
RVDPTNGNSEYDPRFQG

SEQ ID NO: 79 - protein, 17 aa, Synthetic construct
YIYPYNGGAGYNQKFKS

SEQ ID NO: 80 - protein, 17 aa, Synthetic construct
WIFPGSGNTYYNEKFKG

SEQ ID NO: 81 - protein, 16 aa, Synthetic construct
VIWSGGNTEYNAAFRS

SEQ ID NO: 82 - protein, 17 aa, Synthetic construct
VIDASDSKTKYNQKFKG

SEQ ID NO: 83 - protein, 17 aa, Synthetic construct
WIYPGSGYTKYNEKLKG

SEQ ID NO: 84 - protein, 17 aa, Synthetic construct
WIYLGSGHTMYNENFKG

SEQ ID NO: 85 - protein, 17 aa, Synthetic construct
WIFPGSGSTYYNEKFKG

SEQ ID NO: 86 - protein, 17 aa, Synthetic construct
WINTYSGVPTYADDFKG

SEQ ID NO: 87 - protein, 17 aa, Synthetic construct
EILPESGRTNYNEKFKG

SEQ ID NO: 88 - protein, 17 aa, Synthetic construct
AIYPGNADISYNQKFRD

SEQ ID NO: 89 - protein, 17 aa, Synthetic construct
DIEPNNGGTNYNQKFKG

SEQ ID NO: 90 - protein, 17 aa, Synthetic construct
WIFPGSGTTYYNEKFKG

SEQ ID NO: 91 - protein, 17 aa, Synthetic construct
EIDPFDSYTNYNQKFKG

SEQ ID NO: 92 - protein, 17 aa, Synthetic construct
AIDPETGGTAYNQKFKG

SEQ ID NO: 93 - protein, 17 aa, Synthetic construct
DVNPNNGDTSYNQKFKG

SEQ ID NO: 94 - protein, 17 aa, Synthetic construct
TIRDGGSYTYYSDNEKG

SEQ ID NO: 95 - protein, 17 aa, Synthetic construct
IINPYNGDTSYNQKFKD

SEQ ID NO: 96 - protein, 16 aa, Synthetic construct
YISSDGTNNYNPSLRN

SEQ ID NO: 97 - protein, 17 aa, Synthetic construct
TIGGVGGNTYYPDSVKG

SEQ ID NO: 98 - protein, 17 aa, Synthetic construct
TIRGGGGNTYYLDSVKG

SEQ ID NO: 99 - protein, 17 aa, Synthetic construct
TISGGGDKTYYLDILKG

SEQ ID NO: 100 - protein, 17 aa, Synthetic construct
DINPDNGGSTYNQKFKG

SEQ ID NO: 101 - protein, 17 aa, Synthetic construct
IINPYNGGTSYNQKFKG

SEQ ID NO: 102 - protein, 17 aa, Synthetic construct
TISGGGDNTYYPDSVKG

SEQ ID NO: 103 - protein, 17 aa, Synthetic construct
TIRGGGSYTYYLDSVKG

SEQ ID NO: 104 - protein, 17 aa, Synthetic construct
DIYPGNFSPNYNEKFKN

SEQ ID NO: 105 - protein, 17 aa, Synthetic construct
AINPNIGGPSYNQKFKG

SEQ ID NO: 106 - protein, 17 aa, Synthetic construct
DIYPNNGDTNYNQKFKG

SEQ ID NO: 107 - protein, 17 aa, Synthetic construct
VIKPYNGAPSYNQKFKG

SEQ ID NO: 108 - protein, 17 aa, Synthetic construct
TISRGGSFTYYPDSVKG

SEQ ID NO: 109 - protein, 17 aa, Synthetic construct
DIYPGNDSPNYNEKFKN

SEQ ID NO: 110 - protein, 17 aa, Synthetic construct
LIDPSNGGTNYNQKFKD

SEQ ID NO: 111 - protein, 17 aa, Synthetic construct
TFNPNRGGPSYNLKFKG

SEQ ID NO: 112 - protein, 17 aa, Synthetic construct
WIFPGSGSTYFNENFKG

SEQ ID NO: 113 - protein, 17 aa, Synthetic construct
DINPNNGGTSYNQKFKG

SEQ ID NO: 114 - protein, 17 aa, Synthetic construct
SFTMYSDATEYSENFKG

SEQ ID NO: 115 - protein, 17 aa, Synthetic construct
DIHPGNTSPNYNEKFRT

SEQ ID NO: 116 - protein, 17 aa, Synthetic construct
YIRSDSSTIYYTDTVKG

SEQ ID NO: 117 - protein, 17 aa, Synthetic construct
EINPKNGDTNYNQNFKG

SEQ ID NO: 118 - protein, 17 aa, Synthetic construct
YIRSDSSTIYYADTVKG

SEQ ID NO: 119 - protein, 17 aa, Synthetic construct
EINPKNGDTNYSQKFRD

SEQ ID NO: 120 - protein, 17 aa, Synthetic construct
EINPNNGDTNYSQKFRD

SEQ ID NO: 121 - protein, 17 aa, Synthetic construct
EINPKNGDTNYNQNFKA

SEQ ID NO: 122 - protein, 17 aa, Synthetic construct
DINPNNGGTNYNQKFKG

SEQ ID NO: 123 - protein, 17 aa, Synthetic construct
DINPDNGGTSYNQKFKG

SEQ ID NO: 124 - protein, 17 aa, Synthetic construct
EINPNNGDTNFNQKFKG

SEQ ID NO: 125 - protein, 17 aa, Synthetic construct
AINPNDGGTSYNQKFEG

SEQ ID NO: 126 - protein, 17 aa, Synthetic construct
EIYPGTINIYYSERFKG

SEQ ID NO: 127 - protein, 17 aa, Synthetic construct
EIDPSDSYTNYNQKFKG

SEQ ID NO: 128 - protein, 17 aa, Synthetic construct
ANDPKNGGFSYNQRFKG

SEQ ID NO: 129 - protein, 17 aa, Synthetic construct
AINPNNGGTSYNQKFKD

SEQ ID NO: 130 - protein, 17 aa, Synthetic construct
AVNPNTGDISYTQKFKD

SEQ ID NO: 131 - protein, 17 aa, Synthetic construct
AIDPNNGGTNYNQKFKD

SEQ ID NO: 132 - protein, 17 aa, Synthetic construct
AIDPNNDSTNYNQKFKG

SEQ ID NO: 133 - protein, 17 aa, Synthetic construct
GIDPAIGNTVSASKFQD

SEQ ID NO: 134 - protein, 17 aa, Synthetic construct
EIYPGSESPYYSEKFKG

SEQ ID NO: 135 - protein, 17 aa, Synthetic construct
EINPSDGRTNYNEKFKS

SEQ ID NO: 136 - protein, 17 aa, Synthetic construct
AMSPNNGATSYNQKFKG

SEQ ID NO: 137 - protein, 17 aa, Synthetic construct
DIYPGNTFPNYNEKFKG

SEQ ID NO: 138 - protein, 17 aa, Synthetic construct
GIDPAIGNTLYASKFQD

SEQ ID NO: 139 - protein, 17 aa, Synthetic construct
KISNSGGSTNYPDTVKG

SEQ ID NO: 140 - protein, 17 aa, Synthetic construct
AIFPGNGETRDTQKFKG

SEQ ID NO: 141 - protein, 17 aa, Synthetic construct
EINPSDGRTNYNEKFKN

SEQ ID NO: 142 - protein, 17 aa, Synthetic construct
DISNSGGNTYYSDTVKG

SEQ ID NO: 143 - protein, 17 aa, Synthetic construct
DINPDNGAGNYNQKFKG

SEQ ID NO: 144 - protein, 17 aa, Synthetic construct
DINPDNGGTNYNQKFKG

SEQ ID NO: 145 - protein, 17 aa, Synthetic construct
DVNPDNGGTNYNQKFKG

SEQ ID NO: 146 - protein, 17 aa, Synthetic construct
TIVNGGINTYYPDTVKG

SEQ ID NO: 147 - protein, 17 aa, Synthetic construct
TINNGGINTYYPDTVKG

SEQ ID NO: 148 - protein, 17 aa, Synthetic construct
ELSNSGGSFHYPDNVKG

SEQ ID NO: 149 - protein, 17 aa, Synthetic construct
EILPGYISTNYNEKFKD

SEQ ID NO: 150 - protein, 17 aa, Synthetic construct
EILPGSVTTNYNEKFRG

SEQ ID NO: 151 - protein, 17 aa, Synthetic construct
TISDGASYTYYPDNVKG

SEQ ID NO: 152 - protein, 17 aa, Synthetic construct
TITSGDIRTYYPDTVKG

SEQ ID NO: 153 - protein, 17 aa, Synthetic construct
AINPSNGYIGYNQKFKD

SEQ ID NO: 154 - protein, 17 aa, Synthetic construct
DVNPDSNGANYNQKFKG

SEQ ID NO: 155 - protein, 17 aa, Synthetic construct
AINPNNGGTFYNQKFKG

SEQ ID NO: 156 - protein, 17 aa, Synthetic construct
AIDPNNGGTNYNQKFKG

SEQ ID NO: 157 - protein, 16 aa, Synthetic construct
HIWWDDDKYYNPALKS

SEQ ID NO: 158 - protein, 17 aa, Synthetic construct
IINPYNGDTSYNQKFKG

SEQ ID NO: 159 - protein, 17 aa, Synthetic construct
DINPNNGDTTYSQKFMG

SEQ ID NO: 160 - protein, 17 aa, Synthetic construct
AIFPENGDTRYTQKFKG

SEQ ID NO: 161 - protein, 17 aa, Synthetic construct
AIDPKNGATSYNQKFKG

SEQ ID NO: 162 - protein, 10 aa, Synthetic construct
DGGLRGPFDY

SEQ ID NO: 163 - protein, 5 aa, Synthetic construct
GYFDV

SEQ ID NO: 164 - protein, 10 aa, Synthetic construct
DGELRGPFDY

SEQ ID NO: 165 - protein, 5 aa, Synthetic construct
LFFDY

SEQ ID NO: 166 - skipped

SEQ ID NO: 167 - protein, 9 aa, Synthetic construct
FGIYPYFDY

SEQ ID NO: 168 - skipped

SEQ ID NO: 169 - protein, 11 aa, Synthetic construct
YYSGSSYGLDY

SEQ ID NO: 170 - protein, 11 aa, Synthetic construct
YFSGSSYGLDY

SEQ ID NO: 171 - protein, 11 aa, Synthetic construct
EELRRDYGMDY

SEQ ID NO: 172 - protein, 10 aa, Synthetic construct
DSTGLYAMDY

SEQ ID NO: 173 - protein, 8 aa, Synthetic construct
DSFYAMDY

SEQ ID NO: 174 - protein, 9 aa, Synthetic construct
EDYFDRGDC

SEQ ID NO: 175 - protein, 13 aa, Synthetic construct
ELPFTTIIGTKDY

SEQ ID NO: 176 - protein, 6 aa, Synthetic construct
LLFFDY

SEQ ID NO: 177 - protein, 9 aa, Synthetic construct
PLRIYAMDC

SEQ ID NO: 178 - protein, 5 aa, Synthetic construct
LYFDY

SEQ ID NO: 179 - protein, 13 aa, Synthetic construct
RVYYGYDRYFFDY

SEQ ID NO: 180 - protein, 10 aa, Synthetic construct
DGSYDPPFAY

SEQ ID NO: 181 - protein, 14 aa, Synthetic construct
WITTVVATLYYFDY

SEQ ID NO: 182 - protein, 10 aa, Synthetic construct
SGLPYVLMDY

SEQ ID NO: 183 - protein, 10 aa, Synthetic construct
DQVNRGWFTY

SEQ ID NO: 184 - protein, 11 aa, Synthetic construct
DSSNVGNAMDY

SEQ ID NO: 185 - protein, 6 aa, Synthetic construct
GLRYGP

SEQ ID NO: 186 - protein, 11 aa, Synthetic construct
HEDYYYYAMDY

SEQ ID NO: 187 - protein, 11 aa, Synthetic construct
HEDYEWYAMDN

SEQ ID NO: 188 - protein, 11 aa, Synthetic construct
HEDYAWYAMDY

SEQ ID NO: 189 - protein, 10 aa, Synthetic construct
SGPPYVLLDY

SEQ ID NO: 190 - protein, 11 aa, Synthetic construct
DSSNVGNDMDY

SEQ ID NO: 191 - protein, 11 aa, Synthetic construct
HEDYEWYAMDY

SEQ ID NO: 192 - protein, 11 aa, Synthetic construct
HEDYDYYAMDY

SEQ ID NO: 193 - protein, 11 aa, Synthetic construct
SDDYGGYYFDY

SEQ ID NO: 194 - protein, 8 aa, Synthetic construct
GVGLGFPY

SEQ ID NO: 195 - protein, 11 aa, Synthetic construct
SDDFDGYAMDY

SEQ ID NO: 196 - protein, 11 aa, Synthetic construct
PIYYEYDGFAY

SEQ ID NO: 197 - protein, 5 aa, Synthetic construct
GYYDY

SEQ ID NO: 198 - protein, 4 aa, Synthetic construct
GTVY

SEQ ID NO: 199 - protein, 11 aa, Synthetic construct
ADDYDGYYFDY

SEQ ID NO: 200 - protein, 6 aa, Synthetic construct
YYGSNY

SEQ ID NO: 201 - protein, 5 aa, Synthetic construct
VWFAY

SEQ ID NO: 202 - protein, 9 aa, Synthetic construct
GYSGNGFTY

SEQ ID NO: 203 - protein, 5 aa, Synthetic construct
GWGDY

SEQ ID NO: 204 - protein, 12 aa, Synthetic construct
RSPVVVNYAMDY

SEQ ID NO: 205 - protein, 11 aa, Synthetic construct
EGVSSYYAMDY

SEQ ID NO: 206 - protein, 11 aa, Synthetic construct
EGVGSYYAMDY

SEQ ID NO: 207 - protein, 11 aa, Synthetic construct
EGVSSYYGMDS

SEQ ID NO: 208 - protein, 5 aa, Synthetic construct
IWFAY

SEQ ID NO: 209 - protein, 11 aa, Synthetic construct
EGGSSYYAMDY

SEQ ID NO: 210 - protein, 10 aa, Synthetic construct
WVNNDWYFDV

SEQ ID NO: 211 - protein, 10 aa, Synthetic construct
DDGYYDAMDY

SEQ ID NO: 212 - protein, 14 aa, Synthetic construct
SIYYSNYVRYYFDY

SEQ ID NO: 213 - protein, 10 aa, Synthetic construct
WVINDWYFDV

SEQ ID NO: 214 - protein, 10 aa, Synthetic construct
WDSNYWYFDV

SEQ ID NO: 215 - protein, 10 aa, Synthetic construct
WDSDYWYFDV

SEQ ID NO: 216 - protein, 9 aa, Synthetic construct
WSESWYFDV

SEQ ID NO: 217 - protein, 10 aa, Synthetic construct
WDSNDWYFDV

SEQ ID NO: 218 - protein, 10 aa, Synthetic construct
WDSDDWYFDV

SEQ ID NO: 219 - protein, 14 aa, Synthetic construct
ERVHSNTLYYAMDY

SEQ ID NO: 220 - protein, 11 aa, Synthetic construct
SDYSDYWAMDY

SEQ ID NO: 221 - protein, 11 aa, Synthetic construct
NADRAYYTMDY

SEQ ID NO: 222 - protein, 10 aa, Synthetic construct
WDSNSWYFDV

SEQ ID NO: 223 - protein, 14 aa, Synthetic construct
ERVYSNTLYYAMDY

SEQ ID NO: 224 - protein, 10 aa, Synthetic construct
YSWDVYAMDY

SEQ ID NO: 225 - protein, 7 aa, Synthetic construct
FNNYLDY

SEQ ID NO: 226 - protein, 9 aa, Synthetic construct
PDNWDPFVY

SEQ ID NO: 227 - protein, 5 aa, Synthetic construct
LFFDS

SEQ ID NO: 228 - protein, 11 aa, Synthetic construct
HDDFLYYAMDY

SEQ ID NO: 229 - protein, 10 aa, Synthetic construct
HNWDVYAMDY

SEQ ID NO: 230 - protein, 11 aa, Synthetic construct
IVTTYYYFMDY

SEQ ID NO: 231 - protein, 11 aa, Synthetic construct
GSDYSYYAMDY

SEQ ID NO: 232 - protein, 9 aa, Synthetic construct
DELIAPFAY

SEQ ID NO: 233 - protein, 11 aa, Synthetic construct
HDDFHFYAMDY

SEQ ID NO: 234 - protein, 11 aa, Synthetic construct
GEDFDGYAMDY

SEQ ID NO: 235 - protein, 5 aa, Synthetic construct
LFFDN

SEQ ID NO: 236 - protein, 10 aa, Synthetic construct
WDSDSWYFDV

SEQ ID NO: 237 - protein, 7 aa, Synthetic construct
GTYWFTY

SEQ ID NO: 238 - protein, 7 aa, Synthetic construct
FINYVDY

SEQ ID NO: 239 - protein, 11 aa, Synthetic construct
KASQDINKYIA

SEQ ID NO: 240 - protein, 17 aa, Synthetic construct
KSSQSLLNSGNQKNFLA

SEQ ID NO: 241 - protein, 17 aa, Synthetic construct
KSSQSLLNSGNQKNYLA

SEQ ID NO: 242 - protein, 11 aa, Synthetic construct
KASQNVGTAVA

SEQ ID NO: 243 - protein, 11 aa, Synthetic construct
RASQDIGRSLN

SEQ ID NO: 244 - protein, 11 aa, Synthetic construct
KASQSVNKAVV

SEQ ID NO: 245 - protein, 11 aa, Synthetic construct
RASQDIGSSLN

SEQ ID NO: 246 - protein, 17 aa, Synthetic construct
KSSQSLLNSGTQKNYLA

SEQ ID NO: 247 - protein, 11 aa, Synthetic construct
RASQDISNYLN

SEQ ID NO: 248 - protein, 11 aa, Synthetic construct
RASQDIGYSLN

SEQ ID NO: 249 - protein, 11 aa, Synthetic construct
RASENIYSYLA

SEQ ID NO: 250 - protein, 11 aa, Synthetic construct
RTSQDISNFLN

SEQ ID NO: 251 - protein, 10 aa, Synthetic construct
SASSSINYMH

SEQ ID NO: 252 - protein, 11 aa, Synthetic construct
RASQFISNNLH

SEQ ID NO: 253 - protein, 16 aa, Synthetic construct
KSSQSLLDSDGKTYLN

SEQ ID NO: 254 - protein, 11 aa, Synthetic construct
KASQNVGTNVA

SEQ ID NO: 255 - protein, 11 aa, Synthetic construct
KANQDINKYIA

SEQ ID NO: 256 - protein, 10 aa, Synthetic construct
SASSSVSYMH

SEQ ID NO: 257 - protein, 11 aa, Synthetic construct
KASQNVRTAVA

SEQ ID NO: 258 - protein, 11 aa, Synthetic construct
RASENINSYLA

SEQ ID NO: 259 - protein, 12 aa, Synthetic construct
SASSSVSSSYFH

SEQ ID NO: 260 - protein, 12 aa, Synthetic construct
TLSSQHSTYTIE

SEQ ID NO: 261 - protein, 10 aa, Synthetic construct
SANSTVSYIY

SEQ ID NO: 262 - protein, 10 aa, Synthetic construct
SARSSVSYMY

SEQ ID NO: 263 - protein, 10 aa, Synthetic construct
SASSSVNYIY

SEQ ID NO: 264 - protein, 11 aa, Synthetic construct
QTSENIYSYLA

SEQ ID NO: 265 - protein, 10 aa, Synthetic construct
SASSSVSYIY

SEQ ID NO: 266 - protein, 10 aa, Synthetic construct
SASSSVSYMY

SEQ ID NO: 267 - protein, 10 aa, Synthetic construct
RANSSVNYMH

SEQ ID NO: 268 - protein, 11 aa, Synthetic construct
QASQVVSTAVA

SEQ ID NO: 269 - protein, 16 aa, Synthetic construct
RSSQSIVHSNGNTYLE

SEQ ID NO: 270 - protein, 11 aa, Synthetic construct
RASQDIGNNLN

SEQ ID NO: 271 - protein, 11 aa, Synthetic construct
RASQSISSWLA

SEQ ID NO: 272 - protein, 15 aa, Synthetic construct
RASESVDNYGISFMH

SEQ ID NO: 273 - protein, 11 aa, Synthetic construct
RASENIYSHLV

SEQ ID NO: 274 - protein, 17 aa, Synthetic construct
KSSQSLLNSFNQKNFLA

SEQ ID NO: 275 - protein, 11 aa, Synthetic construct
RASENIYSYLV

SEQ ID NO: 276 - protein, 17 aa, Synthetic construct
KSSQSLLSSNNQKSFLA

SEQ ID NO: 277 - protein, 17 aa, Synthetic construct
KSSQSLLNSNNQKNFLA

SEQ ID NO: 278 - protein, 17 aa, Synthetic construct
KSSQSLLNGFNQKNFLA

SEQ ID NO: 279 - protein, 17 aa, Synthetic construct
KSSQSLLSSGNQKNFLA

SEQ ID NO: 280 - protein, 17 aa, Synthetic construct
KSSQSLLNSGIQKNFLA

SEQ ID NO: 281 - protein, 17 aa, Synthetic construct
KSSQSLLSNNNQKNFLA

SEQ ID NO: 282 - protein, 11 aa, Synthetic construct
KASQNVRSAVD

SEQ ID NO: 283 - protein, 11 aa, Synthetic construct
KASQDVRSAVA

SEQ ID NO: 284 - protein, 11 aa, Synthetic construct
KASQNVRTAVD

SEQ ID NO: 285 - protein, 11 aa, Synthetic construct
KASQNVRAAVD

SEQ ID NO: 286 - protein, 11 aa, Synthetic construct
KASQNVRIAVD

SEQ ID NO: 287 - protein, 11 aa, Synthetic construct
KASEDIYNRLA

SEQ ID NO: 288 - protein, 15 aa, Synthetic construct
RASKSVSISGYSYMH

SEQ ID NO: 289 - protein, 11 aa, Synthetic construct
KASQNVRSAVA

SEQ ID NO: 290 - protein, 11 aa, Synthetic construct
RASQSVSSNLA

SEQ ID NO: 291 - protein, 17 aa, Synthetic construct
KSSQSLLNSFNQRNFLA

SEQ ID NO: 292 - protein, 11 aa, Synthetic construct
KASQIVRTAVD

SEQ ID NO: 293 - protein, 17 aa, Synthetic construct
KSSQSLLNGFNQRNFLA

SEQ ID NO: 294 - protein, 11 aa, Synthetic construct
KASEDIYARLA

SEQ ID NO: 295 - protein, 17 aa, Synthetic construct
RSSQSLLNSGNQKNYLA

SEQ ID NO: 296 - protein, 10 aa, Synthetic construct
SASSSVSYMF

SEQ ID NO: 297 - protein, 11 aa, Synthetic construct
RASENVNSYLA

SEQ ID NO: 298 - protein, 10 aa, Synthetic construct
SASSSVTYMH

SEQ ID NO: 299 - protein, 17 aa, Synthetic construct
KSSQSLLNIFNQKNFLA

SEQ ID NO: 300 - protein, 11 aa, Synthetic construct
KASQDVGTAVA

SEQ ID NO: 301 - protein, 10 aa, Synthetic construct
SASSSVSYLY

SEQ ID NO: 302 - protein, 10 aa, Synthetic construct
SASSSVNYMF

SEQ ID NO: 303 - protein, 11 aa, Synthetic construct
KASENVRAAVD

SEQ ID NO: 304 - protein, 16 aa, Synthetic construct
RSSQSIEHSNGNTYLQ

SEQ ID NO: 305 - protein, 10 aa, Synthetic construct
SASSSVNNIH

SEQ ID NO: 306 - protein, 11 aa, Synthetic construct
KASQNIRSAVA

SEQ ID NO: 307 - protein, 7 aa, Synthetic construct
YTSTLHP

SEQ ID NO: 308 - protein, 7 aa, Synthetic construct
YTSTLQP

SEQ ID NO: 309 - protein, 7 aa, Synthetic construct
GTSTRES

SEQ ID NO: 310 - protein, 7 aa, Synthetic construct
YTSTLQA

SEQ ID NO: 311 - protein, 7 aa, Synthetic construct
GASTRES

SEQ ID NO: 312 - protein, 7 aa, Synthetic construct
SASNRYT

SEQ ID NO: 313 - protein, 7 aa, Synthetic construct
ATSRLDS

SEQ ID NO: 314 - protein, 7 aa, Synthetic construct
YASNRYT

SEQ ID NO: 315 - protein, 7 aa, Synthetic construct
YTSRLHS

SEQ ID NO: 316 - protein, 7 aa, Synthetic construct
NAKTLAE

SEQ ID NO: 317 - protein, 7 aa, Synthetic construct
FTSTLQS

SEQ ID NO: 318 - protein, 7 aa, Synthetic construct
DTSKLAS

SEQ ID NO: 319 - protein, 7 aa, Synthetic construct
YASQSIS

SEQ ID NO: 320 - protein, 7 aa, Synthetic construct
LVSKLDS

SEQ ID NO: 321 - protein, 7 aa, Synthetic construct
SASYRYS

SEQ ID NO: 322 - protein, 7 aa, Synthetic construct
YTSTLQS

SEQ ID NO: 323 - protein, 7 aa, Synthetic construct
STSNLAS

SEQ ID NO: 324 - protein, 7 aa, Synthetic construct
LASNRHT

SEQ ID NO: 325 - protein, 7 aa, Synthetic construct
NTKTLTE

SEQ ID NO: 326 - protein, 7 aa, Synthetic construct
YSSRLHS

SEQ ID NO: 327 - protein, 7 aa, Synthetic construct
GSHRTGD

SEQ ID NO: 328 - protein, 7 aa, Synthetic construct
DTSNLAS

SEQ ID NO: 329 - protein, 7 aa, Synthetic construct
NTQTLAE

SEQ ID NO: 330 - protein, 7 aa, Synthetic construct
ATSNLAS

SEQ ID NO: 331 - protein, 7 aa, Synthetic construct
SASFRYS

SEQ ID NO: 332 - protein, 7 aa, Synthetic construct
KVSNRFS

SEQ ID NO: 333 - protein, 7 aa, Synthetic construct
ATSSLDS

SEQ ID NO: 334 - protein, 7 aa, Synthetic construct
TVSNRLS

SEQ ID NO: 335 - protein, 7 aa, Synthetic construct
KASTLES

SEQ ID NO: 336 - protein, 7 aa, Synthetic construct
RASNLES

SEQ ID NO: 337 - protein, 7 aa, Synthetic construct
NGKILAE

SEQ ID NO: 338 - protein, 7 aa, Synthetic construct
FASTRES

SEQ ID NO: 339 - protein, 7 aa, Synthetic construct
SASNRHT

SEQ ID NO: 340 - protein, 7 aa, Synthetic construct
LASSRHT

SEQ ID NO: 341 - protein, 7 aa, Synthetic construct
SSSNRHT

SEQ ID NO: 342 - protein, 7 aa, Synthetic construct
GTTSLEI

SEQ ID NO: 343 - protein, 7 aa, Synthetic construct
LASNLES

SEQ ID NO: 344 - protein, 7 aa, Synthetic construct
GASTRAT

SEQ ID NO: 345 - protein, 7 aa, Synthetic construct
FASTRDS

SEQ ID NO: 346 - protein, 7 aa, Synthetic construct
SASTRHT

SEQ ID NO: 347 - protein, 7 aa, Synthetic construct
GASTRQS

SEQ ID NO: 348 - protein, 7 aa, Synthetic construct
NAETLVE

SEQ ID NO: 349 - protein, 7 aa, Synthetic construct
DTSKLTS

SEQ ID NO: 350 - protein, 7 aa, Synthetic construct
GATSLET

SEQ ID NO: 351 - protein, 7 aa, Synthetic construct
NAQTLAE

SEQ ID NO: 352 - protein, 7 aa, Synthetic construct
WASTRHT

SEQ ID NO: 353 - protein, 7 aa, Synthetic construct
SASSRHT

SEQ ID NO: 354 - protein, 7 aa, Synthetic construct
NAKTLTE

SEQ ID NO: 355 - protein, 7 aa, Synthetic construct
DTTKLTS

SEQ ID NO: 356 - protein, 7 aa, Synthetic construct
LTSNRHT

SEQ ID NO: 357 - protein, 8 aa, Synthetic construct
LQYDYLLT

SEQ ID NO: 358 - protein, 8 aa, Synthetic construct
LQYDNLHT

SEQ ID NO: 359 - protein, 9 aa, Synthetic construct
QNDHSYPWT

SEQ ID NO: 360 - protein, 8 aa, Synthetic construct
LQYDNLLT

SEQ ID NO: 361 - protein, 9 aa, Synthetic construct
QNAHSSPYT

SEQ ID NO: 362 - protein, 8 aa, Synthetic construct
QQYSSYRT

SEQ ID NO: 363 - protein, 9 aa, Synthetic construct
LQYASFPYT

SEQ ID NO: 364 - protein, 9 aa, Synthetic construct
QQDYSSPWT

SEQ ID NO: 365 - protein, 9 aa, Synthetic construct
LQYASSPYT

SEQ ID NO: 366 - protein, 9 aa, Synthetic construct
QQGNMFPPT

SEQ ID NO: 367 - protein, 9 aa, Synthetic construct
QHHYGTPYT

SEQ ID NO: 368 - protein, 8 aa, Synthetic construct
LQYDYLYT

SEQ ID NO: 369 - protein, 9 aa, Synthetic construct
QQGYMLPPT

SEQ ID NO: 370 - protein, 9 aa, Synthetic construct
QQGNTLPPT

SEQ ID NO: 371 - protein, 8 aa, Synthetic construct
LQYSSYLT

SEQ ID NO: 372 - protein, 8 aa, Synthetic construct
QQYSTYLT

SEQ ID NO: 373 - protein, 9 aa, Synthetic construct
HQRSSYPFT

SEQ ID NO: 374 - protein, 9 aa, Synthetic construct
QQSNSWPHT

SEQ ID NO: 375 - protein, 9 aa, Synthetic construct
WQGTHFPLT

SEQ ID NO: 376 - protein, 9 aa, Synthetic construct
QQYNSRPLT

SEQ ID NO: 377 - protein, 9 aa, Synthetic construct
QNDHSYPFT

SEQ ID NO: 378 - protein, 8 aa, Synthetic construct
LQYDHLLT

SEQ ID NO: 379 - protein, 9 aa, Synthetic construct
QQRSSYPPT

SEQ ID NO: 380 - protein, 8 aa, Synthetic construct
LQYDNLYT

SEQ ID NO: 381 - protein, 9 aa, Synthetic construct
LQHWNYPLT

SEQ ID NO: 382 - protein, 9 aa, Synthetic construct
QHHYGTPLT

SEQ ID NO: 383 - protein, 9 aa, Synthetic construct
HQHHRSPLT

SEQ ID NO: 384 - protein, 9 aa, Synthetic construct
QQGYTLPRT

SEQ ID NO: 385 - protein, 9 aa, Synthetic construct
QQGNTLPRT

SEQ ID NO: 386 - protein, 9 aa, Synthetic construct
GVGDINNYI

SEQ ID NO: 387 - protein, 9 aa, Synthetic construct
QQWSSFPFT

SEQ ID NO: 388 - protein, 9 aa, Synthetic construct
QQWSSYPLT

SEQ ID NO: 389 - protein, 8 aa, Synthetic construct
LQYDNLYM

SEQ ID NO: 390 - protein, 9 aa, Synthetic construct
QHHYGVPLT

SEQ ID NO: 391 - protein, 9 aa, Synthetic construct
QQWTSYPLT

SEQ ID NO: 392 - protein, 9 aa, Synthetic construct
QQWTSNPLT

SEQ ID NO: 393 - protein, 9 aa, Synthetic construct
QQHYRTPYT

SEQ ID NO: 394 - protein, 9 aa, Synthetic construct
FQGSHVPRT

SEQ ID NO: 395 - protein, 9 aa, Synthetic construct
QNDHSYPHT

SEQ ID NO: 396 - protein, 9 aa, Synthetic construct
LQYASSPVT

SEQ ID NO: 397 - protein, 9 aa, Synthetic construct
QQWTNNPLT

SEQ ID NO: 398 - protein, 9 aa, Synthetic construct
FQTSHVPPT

SEQ ID NO: 399 - protein, 8 aa, Synthetic construct
QQYNTYWT

SEQ ID NO: 400 - protein, 9 aa, Synthetic construct
QNAHSYPFT

SEQ ID NO: 401 - protein, 10 aa, Synthetic construct
QQSNKDPMYT

SEQ ID NO: 402 - protein, 9 aa, Synthetic construct
QNDHGYPLT

SEQ ID NO: 403 - protein, 9 aa, Synthetic construct
QHHYGSPIT

SEQ ID NO: 404 - protein, 9 aa, Synthetic construct
QQHHSTPPT

SEQ ID NO: 405 - protein, 9 aa, Synthetic construct
LQYASSPPT

SEQ ID NO: 406 - protein, 9 aa, Synthetic construct
QHHYGSPLT

SEQ ID NO: 407 - protein, 9 aa, Synthetic construct
QQHYSTPPT

SEQ ID NO: 408 - protein, 9 aa, Synthetic construct
QNAHSSPFT

SEQ ID NO: 409 - protein, 9 aa, Synthetic construct
LQHWNYPYT

SEQ ID NO: 410 - protein, 9 aa, Synthetic construct
LQYTSSPWT

SEQ ID NO: 411 - protein, 8 aa, Synthetic construct
LQYDNLWT

SEQ ID NO: 412 - protein, 9 aa, Synthetic construct
LQHWTYPYT

SEQ ID NO: 413 - protein, 9 aa, Synthetic construct
LQHWISPYT

SEQ ID NO: 414 - protein, 9 aa, Synthetic construct
LQHWNSPYT

SEQ ID NO: 415 - protein, 9 aa, Synthetic construct
QQYWSTPWT

SEQ ID NO: 416 - protein, 9 aa, Synthetic construct
QHSRELPPT

SEQ ID NO: 417 - protein, 9 aa, Synthetic construct
LQHWNYPWT

SEQ ID NO: 418 - protein, 9 aa, Synthetic construct
HQYNNWPRT

SEQ ID NO: 419 - protein, 9 aa, Synthetic construct
QNDHSYPYT

SEQ ID NO: 420 - protein, 8 aa, Synthetic construct
QHHYGDPT

SEQ ID NO: 421 - protein, 9 aa, Synthetic construct
QQWISNPYT

SEQ ID NO: 422 - protein, 9 aa, Synthetic construct
QQHWSTPWT

SEQ ID NO: 423 - protein, 9 aa, Synthetic construct
QNAHTSPYT

SEQ ID NO: 424 - protein, 8 aa, Synthetic construct
QHHYGNPT

SEQ ID NO: 425 - protein, 9 aa, Synthetic construct
QQRSSYPWT

SEQ ID NO: 426 - protein, 9 aa, Synthetic construct
QQYNSYPWT

SEQ ID NO: 427 - protein, 9 aa, Synthetic construct
FQGSHVPWT

SEQ ID NO: 428 - protein, 9 aa, Synthetic construct
QQGHALPRT

SEQ ID NO: 429 - protein, 9 aa, Synthetic construct
QQWNINPYT

SEQ ID NO: 430 - protein, 119 aa, Synthetic construct
QVHLQQSGPELVKPGASLKISCKASGYTFTDYYLNWVKQRPGQGLEWIGWIFPGSESTFYNEKFKGKATLTVDKSSSTAYMLLNSLTSEDSAVYFCTRDGGLRGPFDYWGQGTTLTVSS

SEQ ID NO: 431 - protein, 106 aa, Synthetic construct
DIQLTQSPSSLSASLGGKVTITCKASQDINKYIAWCQHKPGKGPRLLIHYTSTLHPGIPSRFSGSGSGRDYSFSISNLEPEDSATYYCLQYDYLLTFGGGTKLEIK

SEQ ID NO: 432 - protein, 119 aa, Synthetic construct
QVQLQQSGPELVKPGASVKISCRSSGYTFTDYYINWVKQRPGQGLEWIGWIFPGSDYTYYNEKFKGKATLTVDKSSTTAYMLLSSLTSEDSAVYFCARDGGLRGPFDYWGQGTTLTVSS

SEQ ID NO: 433 - protein, 106 aa, Synthetic construct
DIQMTQSPSSLSASLGGKVTITCKASQDINKYIAWYQQKPGKGPRLLIHYTSTLQPGIPSRFSGSGSGRNSSFSISNLEPEDIATYYCLQYDNLHTFGGGTKLEIK

SEQ ID NO: 434 - protein, 114 aa, Synthetic construct
EVQLQQSGPELVKPGASVKISCKASGYTFTDYFMNWVKQSHGKSLEWIGDIIPNNDSPNYNQKFKGKATLTVDKSSNTAYMELRSLTSEDSAVYYCASGYFDVWGTGTTVTVSS

SEQ ID NO: 435 - protein, 113 aa, Synthetic construct
DIVMTQSPSSLSVSAGEKVTMSCKSSQSLLNSGNQKNFLAWYQQKPGQPPKLLIYGTSTRESGVPDRFTGSGSGTDFTLTISSVQAEDLAVYYCQNDHSYPWTFGGGTKLEIK

SEQ ID NO: 436 - protein, 119 aa, Synthetic construct
QVHLHQSGPELVKPGASVKISCKASGYTFTAYYINWVKQRPGQGLEWIGWIFPGSDSTYYNEKFKGRATLTVDKSSSTAYMLLNSLTSEDSAVYFCARDGELRGPFDYWGQGTTLTVSS

SEQ ID NO: 437 - protein, 106 aa, Synthetic construct
DIQMTQSPSSLSASLGGKVTITCKASQDINKYIAWYQHKPGKSPRLLIHYTSTLQAGIPSRFSGSGSGRDYSFSISNLEPEDSATYYCLQYDNLLTFGGGTKLEIK

SEQ ID NO: 438 - protein, 114 aa, Synthetic construct
EVQLQQSGPELVKPGASVKISCKASGYTLTDYYMNWVKQSHGKSLEWIGDINPNNGGTNFNQKFKGKATLTIDKSSSTTYMELRSLTSEDSAVYYCASLFFDYWGQGTTLTVSS

SEQ ID NO: 439 - protein, 113 aa, Synthetic construct
DIVMTQSPSSLSVSAGEKVTMSCKSSQSLLNSGNQKNYLAWYQQKPGQPPKLLIYGASTRESGVPDRFTGSGSGTDFTLTISSVQAEDLALYYCQNAHSSPYTFGGGTKLEIK

SEQ ID NO: 440 - protein, 106 aa, Synthetic construct
DIVMTQSQKFMSTTVGDRVSITCKASQNVGTAVAWYQQKPGQSPKLLIYSASNRYTGVPDRFTGSGSGTDFTLTISNMQSEDLADYFCQQYSSYRTFGGGTKLEIK

SEQ ID NO: 441 - protein, 112 aa, Synthetic construct
EVQLVASGGGLVKPGGSLKLSCAASGFTFSDYYMFWVRQTPEKRLEWVATISDGGGYIYYPDSVKGRFTISRDNDRNSLYLQMSSLKSEDTAIYYCGREDFWGQGTSVTVSS

SEQ ID NO: 442 - protein, 107 aa, Synthetic construct
DIQMTQSPSSLSASLGERVSLTCRASQDIGRSLNWLQQEPDGSVRRLIYATSRLDSGVPKRFSGSRSGSDYSLTISSLESEDFVDYYCLQYASFPYTFGGGTKLEIK

SEQ ID NO: 443 - protein, 118 aa, Synthetic construct
EVQLQQSGAELVKPGASVKLSCTASGFNIKDIYMHWLKQRPEQGLEWIGRIDPTNGNSEYDPRFRGKATLTADTSSNIAYLQLSSLTSEDTAVYYCARFGIYPYFDYWGQGTTLTVSS

SEQ ID NO: 444 - protein, 107 aa, Synthetic construct
GIVMTQTPKFLLVSAGDRVTITCKASQSVNKAVVWYQQKPGQSPKLLISYASNRYTGVPDRFTGSGYGTDFTFSISTVQAEDLAVYFCQQDYSSPWTFGGGTKLEIK

SEQ ID NO: 445 - protein, 112 aa, Synthetic construct
EVELVESGGGLVKPGGSLKLSCAASGFTFSDSYMCWVRQTPEKRLEWVATISDGGGLTYYPDSVKGRFTISRDNDRNNLYLQMDSLKSEDTAVYYCGREDLWGQGTSVIVSS

SEQ ID NO: 446 - protein, 107 aa, Synthetic construct
DIQMTQSPSSLSASLGERVSLTCRASQDIGSSLNWLQQEPDGTIKRLIYATSRLDSGVPKRFSGSRSGSDYSLTISSLESEDFVDYYCLQYASSPYTFGGGTKLEIK

SEQ ID NO: 447 - protein, 114 aa, Synthetic construct
EVQLQQSGPELVKPGASVKISCKASGYTFTDYFMNWVRQSHGKSLEWIGDIHPNNGSPNYNQKFKGKATLTVGKSSSTAYMELRSLTSEDSAVYYCATGYFDVWGTGTTVTVSS

SEQ ID NO: 448 - protein, 113 aa, Synthetic construct
DIVMTQSPSSLSVSAGEKVTMSCKSSQSLLNSGNQKNYLAWYQQKPGQPPKLLIYGASTRESGVPDRFTGSGSGTDFTLTISSVQAEDLAVYYCQNDHSYPWTFGGGTKLEIK

SEQ ID NO: 449 - protein, 112 aa, Synthetic construct
EVQLVASGGGLVKPGGSLKLSCAASGFTFSDYYMYWVRQTPEKRLEWVATISDGGGYTYYPDSVKGRFTISRDNDRNSLYLQMSSLKSEDTAMYYCGREDLWGQGTSVTVSS

SEQ ID NO: 450 - protein, 107 aa, Synthetic construct
DIQMTQSPSSLSASLGERVSLTCRASQDIGSSLNWLQQEPDGTVKRLIYATSRLDSGVPKRFSGSRSGSDYSLTISSLESEDFVDYYCLQYASFPYTFGGGTKLEIK

SEQ ID NO: 451 - protein, 114 aa, Synthetic construct
EVQLQQSGPELVKPGASVKISCKASGYTFTDYFMNWVKQSHGKSLEWIGDINPNNGSPNYNQKFKGRATLTVDKSSSTAYMELRSLTSEDSAVYYCASGYFDVWGTGTTVTVSS

SEQ ID NO: 452 - protein, 113 aa, Synthetic construct
DIVMTQSPSSLSVSAGEKVTMSCKSSQSLLNSGTQKNYLAWYQQKPGQPPKLLIYGASTRESGVPDRFTGSGSGTDFTLTISSVQAEDLAVYYCQNDHSYPWTFGGGTKLEIK

SEQ ID NO: 453 - protein, 120 aa, Synthetic construct
QVQLQQPGAELVRPGTSVKLSCKASGNTFTSYWMHWVKQRPGQGHEWIGVIDASDSNTKYNQKFKGKATLTVDTSSSTAYMQLSSLTSEDSAVYYCARYYSGSSYGLDYWGQGTTLTVSS

SEQ ID NO: 454 - protein, 107 aa, Synthetic construct
DIQMTQTASSLSASLGDRVTISCRASQDISNYLNWYQQKPDGTVKLLIYYTSRLHSGVPSRFSGSGSGTDFSLTITHLEQEDIASYFCQQGNMFPPTFGGGTKLEIK

SEQ ID NO: 455 - protein, 120 aa, Synthetic construct
QVQLQQPGAELVRPGTSVKLSCKASGNTFTSYWMHWVKQRPGQGHEWIGVIDASDSNTKYNQKFKGKATLTVDTSSSTAYMQLSSLTSEDSAVYYCARYFSGSSYGLDYWGQGTTLTVSS

SEQ ID NO: 456 - protein, 107 aa, Synthetic construct
DIQMTQTASSLSASLGDRVTISCRASQDISNYLNWYQQKPDGTVKLLIYYTSRLHSGVPSRFSGSGSGTDYSLTITNLEQEDIASYFCQQGNMFPPTFGGGTKLEIK

SEQ ID NO: 457 - protein, 112 aa, Synthetic construct
EVQLVESGGGLVKPGGSLKLSCAASGFTFSDYYMYWVRQTPEKRLEWVATISDGGGFIYYPDSVKGRFTISRDNDRNSLYLLMSSLKSEDTAMYFCGREDLWGQGTSVTVSS

SEQ ID NO: 458 - protein, 107 aa, Synthetic construct
DIQMTQSPSSLSASLGERVSLTCRASQDIGRSLNWLQQGPDGTVKRLIYATSRLDSGVPTRFSGSRSGSDYSLTISSLESEDFVDYYCLQYASFPYTFGGGTKLEIK

SEQ ID NO: 459 - protein, 112 aa, Synthetic construct
EVQLVESGGGLVKPGGSLKLSCAASGFTFSDYYMYWVRQTPEKRLEWVATISDAGGYTYYPDSVKGRFTISRDNARNSLYLQMSSLKSEDTAMYFCGREDLWGQGTSVTVSS

SEQ ID NO: 460 - protein, 107 aa, Synthetic construct
DIQMTQSPSSLSASLGERVSLTCRASQDIGYSLNWLQQEPDGSVRRLIYATSRLDSGVPKRFSGSRSGSDYSLTISSLESEDFVDYYCLQYASFPYTFGGGTKLEIK

SEQ ID NO: 461 - protein, 112 aa, Synthetic construct
EVQLVESGGGLVKPGGSLKLSCAASGFTFSDSYMCWVRQTPEKRLEWVATISDAGGYTYYPDSVKGRFTISRDNDRNNLYLQMSGLKSEDTAVYYCGREDLWGQGTSVTVSS

SEQ ID NO: 462 - protein, 107 aa, Synthetic construct
DIQMTQSPSSLSASLGERVSLTCRASQDIGRSLNWLQQEPDGTIKRLIYATSRLDSGVPKRFSGSRSGSDYSLTISSLESEDFVDYYCLQYASSPYTFGGGTKLEIK

SEQ ID NO: 463 - protein, 118 aa, Synthetic construct
EVQLQQSGAELVKPGASVKLSCTASGFNIKDIYMHWLKQRPEQGLEWIGRVDPTNGNSEYDPRFQGKATLTADTSSNIAYLQLSSLTSEDTAVYYCARFGIYPYFDYWGQGTTLTVSS

SEQ ID NO: 464 - protein, 107 aa, Synthetic construct
SIVMTQTPKFLLVSAGDRVTITCKASQSVNKAVVWYQQKPGQSPKLLINYASNRYTGVPDRFTGSGYGTDFTFSISTVQAEDLAVYFCQQDYSSPWTFGGGTKLEIK

SEQ ID NO: 465 - protein, 120 aa, Synthetic construct
EVQLQQSGPEPVKPGASVKISCKASGYTFTDYNIHWVRQSHGKSLEWIGYIYPYNGGAGYNQKFKSKATLTVDSSSSTAYMELRSLTSEDSAVYYCAREELRRDYGMDYWGQGTSVTVSS

SEQ ID NO: 466 - protein, 107 aa, Synthetic construct
DIQMTQSPASLSASVGETVTITCRASENIYSYLAWYQQKQGKSPQLLVYNAKTLAEGVPSRFSGSGSGTQFSLKINSLQPEDFGSYYCQHHYGTPYTFGGGTKLETK

SEQ ID NO: 467 - protein, 119 aa, Synthetic construct
QVQLQQSGPELVKPGTSVKISCKASGYTFTDYYINWVKQRPGQGLEWIGWIFPGSGNTYYNEKFKGRATLTVDKSSSTAYMLLSSLTSEDSAVYFCARDGGLRGPFDYWGQGTTLTVSS

SEQ ID NO: 468 - protein, 106 aa, Synthetic construct
DIQMTQSPSSLSASLGGKVTITCKASQDINKYIAWFQHKPGKGPRLLIHFTSTLQSGIPSRFSGSGSGGDYSFSISNLEPEDIATYYCLQYDYLYTFGGGTTLEIK

SEQ ID NO: 469 - protein, 118 aa, Synthetic construct
QVQLKQSGPGLVQPSQNLSITCTVSGFSLTGYGINWVRQSPGKGLEWLGVIWSGGNTEYNAAFRSRLSISKDTSKSQVFLKMNSLQADDTAIYSCARDSTGLYAMDYWGPGTSVTVSS

SEQ ID NO: 470 - protein, 107 aa, Synthetic construct
DLQMTQTTSSLSASLGDRVTISCRTSQDISNFLNWYQQKPDGPLKLLIYYTSRLHSGVPSRFSGSGSGTDYSLTISNLEQEDIATYFCQQGYMLPPTFGGGTKLEIK

SEQ ID NO: 471 - protein, 120 aa, Synthetic construct
QVQLQQPGAELVRPGTSVKLSCKASGNTFTSYWMHWVKQRPGQGHEWIGVIDASDSKTKYNQKFKGKATLTVDTSSSTAYMQLSSLTSEDSAVYYCARYYSGSSYGLDYWGQGTTLTVSS

SEQ ID NO: 472 - protein, 107 aa, Synthetic construct
DIQMTQTASSLSASLGDRVTISCRASQDISNYLNWYQQKPDGTVKLLIYYTSRLHSGVPSRFSGSGSGTDYSLTISNLEQEDIATYFCQQGNTLPPTFGGGTKLEIK

SEQ ID NO: 473 - protein, 117 aa, Synthetic construct
QIQLQQSGPELVKPGPSVKISCKASGYTFTDYYINWVKQRPGQGLEWIGWIYPGSGYTKYNEKLKGRATLTVDTSSSTAYMQLSSLTSEDSAVYFCARDSFYAMDYWGQGTSVTVSS

SEQ ID NO: 474 - protein, 106 aa, Synthetic construct
DIVMTQSQKFMSTTVGDRVSITCKASQNVGTAVAWYQQKPGQSPKLLIYSASNRYTGVPDRFTGSGSGTDFTLTITNMQSEDLADYFCLQYSSYLTFGAGTKLELK

SEQ ID NO: 475 - protein, 117 aa, Synthetic construct
QIQLQQSGPELVKPGASVKISCKASGYTFTDYYIAWVKQRPGQGLEWIGWIYLGSGHTMYNENFKGKATLTVDTSSSTAYMQLSSLTSEDSAVYFCARDSFYAMDYWGQGTSVTVSS

SEQ ID NO: 476 - protein, 106 aa, Synthetic construct
DIVMTQSQKFMSTTVGDRVSITCKASQNVGTAVAWYQQKPGQSPKLLIYSASNRYTGVPDRFTGSGSGTDFTLTISNMQSEDLADYFCQQYSTYLTFGAGTKLELK

SEQ ID NO: 477 - protein, 118 aa, Synthetic construct
QVQLQQSGPELVKPGASVKISCKASGYTFTDYYINWVKQRPGQGLEWIGWIFPGSGSTYYNEKFKGKATPTVDKYSSTAYMLLSSLTSEDSAVYFCAREDYFDRGDCWGQGTSVTVSS

SEQ ID NO: 478 - protein, 106 aa, Synthetic construct
QIVLTQSPAIMSASPGEKVTMTCSASSSINYMHWYQQKPGTSPKRWIYDTSKLASGVPARFSGSGSGTSYSLTISSMEAEDAATYYCHQRSSYPFTFGSGTKLEIK

SEQ ID NO: 479 - protein, 122 aa, Synthetic construct
QIQLVQSGPELKKPGETVKISCKASGYTFTTYGMSWVKQAPGKGLKWMGWINTYSGVPTYADDFKGRFAFSLETSASNAYLQINNLKNEDTATYFCARELPFTTIIGTKDYWGQGTTLTVSS

SEQ ID NO: 480 - protein, 107 aa, Synthetic construct
DIVLIQSPATLSVTPGDSVSLSCRASQFISNNLHWYQQKSHESPRLLIKYASQSISGIPSRFSGGGSGTDFTLTVNSVETEDFGMYFCQQSNSWPHTFGGGTKLEIK

SEQ ID NO: 481 - protein, 115 aa, Synthetic construct
QVQLQQSGAELMKPGASVKLSCKATGYTFTGYWIEWVKQRPGHGLEWIGEILPESGRTNYNEKFKGKATFTADTSSNTAYMQLSSLTTEDSAIYYCASLLFFDYWGQGTTLTVSS

SEQ ID NO: 482 - protein, 112 aa, Synthetic construct
DVVLTQTPLTLTVTIGQPASISCKSSQSLLDSDGKTYLNWLLQRPGQSPKRLIYLVSKLDSGVPDRFTGSGSGTDFTLKISRVEAEDLGVYYCWQGTHFPLTFGAGTKLELK

SEQ ID NO: 483 - protein, 118 aa, Synthetic construct
QAYLQQSGAELVRPGASVKMSCKASGYTFTSYNIHWVKQTPRQGLEWIGAIYPGNADISYNQKFRDKATLTVDKSSSTAYMQLSSLTSEDSAVYFCAKPLRIYAMDCWGQGTSVTVSS

SEQ ID NO: 484 - protein, 107 aa, Synthetic construct
DIVMTQSQKFMSTSVGDRVSVTCKASQNVGTNVAWYQQKPGQSPKALIYSASYRYSGVPDRFTGSGSGTDFTLTISNVQSEDLADYFCQQYNSRPLTFGGGTKLEIK

SEQ ID NO: 485 - protein, 114 aa, Synthetic construct
EVQLQQSGPELVKPGASVKISCKASGNTFTDYYINWVKQSHGKSLEWIGDIEPNNGGTNYNQKFKGKATLTVDKSSSTAYMELRSLTSEDSAIYYCATLYFDYWGQGTTLTVSS

SEQ ID NO: 486 - protein, 113 aa, Synthetic construct
DIVMTQSPSSLSVSAGEKVTMSCKSSQSLLNSGNQKNYLAWYQQKPGQPPKLLIYGASTRESGVPDRFTGSGSGTDFTLTISSVQAEDLAVYYCQNDHSYPFTFGSGTKLEIK

SEQ ID NO: 487 - protein, 120 aa, Synthetic construct
QVQLQQPGAELVRPGTSVKLSCKASGNTFTTYWMHWVKQRPGQGHEWIGVIDASDSNTKYNQKFKGKATLTVDTSSSTAYMQLSSLTSEDSAVYYCARYYSGSSYGLDYWGQGTTLTVSS

SEQ ID NO: 488 - protein, 119 aa, Synthetic construct
QVQLQQSGPELMKPGASLKISCKASGYTFTDSYINWVKQRPGQGLEWIGWIFPGSGSTYYNEKFKGTATLTVDKSSSTAYMLLSSLTSEDSAAYFCARDGGLRGPFDYWGQGTTLTVSS

SEQ ID NO: 489 - protein, 106 aa, Synthetic construct
DIQMTQSPSSLSASLGGKVTITCKASQDINKYIAWYQHKPGKGPRLLIHYTSTLQSGIPSRFSGSGSGRDYFFSISNLESEDIATYYCLQYDHLLTFGGGTKLEIK

SEQ ID NO: 490 - protein, 119 aa, Synthetic construct
QVHLQQSGPDLVKPGVSVKISCKASGYTFTDYYINWVKQRPGQGLEWIGWIFPGSGTTYYNEKFKGKATLTVDKSSSTAYMLLSSLTSEDSAVYFCARDGGLRGPFDYWGQGTTLTVSS

SEQ ID NO: 491 - protein, 106 aa, Synthetic construct
DIQMTQSPSSLSASLGGKVTITCKANQDINKYIAWYQYKPGKGPRLLIHYTSTLQPDIPSRFSGSGSGRDFSFSISNLEPEDIATYYCLQYDYLYTFGGGTKLEIK

SEQ ID NO: 492 - protein, 122 aa, Synthetic construct
QVQLQQPGAELVKPGASVKLSCKASGYSFTSYWMQWIKQRPGQGLEWIGEIDPFDSYTNYNQKFKGKATLTVDTSSSTAYMQLSSLTSEDSAVYYCASRVYYGYDRYFFDYWGQGTTLTVSS

SEQ ID NO: 493 - protein, 119 aa, Synthetic construct
QVQLQQSGPELVKPGASVKISCKASGYTFTDYYINWVKQRPGQGLEWIGWIFPGSGSTYYNEKFKGKATLTVDKSSSTAYMLLSSLTSEDSAVYFCAPDGSYDPPFAYWGLGTLVTVSA

SEQ ID NO: 494 - protein, 106 aa, Synthetic construct
QIVLTQSPAIMSASPGEKVTITCSASSSVSYMHWFQQKPGTSPKLWIYSTSNLASGVPARFSGSGSGTSYSLTISRMEAEDAATYYCQQRSSYPPTFGAGTKLELK

SEQ ID NO: 495 - protein, 106 aa, Synthetic construct
DIQMTQSPSSLSASLGGKVTITCKASQDINKYIAWYQHKPGKGPRLLIHYTSTLQPGIPSRFSGSGSGRDYSFSISNLEPEDIATYYCLQYDNLYTFGGGTKLEIK

SEQ ID NO: 496 - protein, 123 aa, Synthetic construct
QVQLQQSGAELVRPGASVTLSCKASGYTFTDYEMHWVKQTPVHGLEWIGAIDPETGGTAYNQKFKGKAILTADKSSSTAYMELRSLTSEDSAVYYCTRWITTVVATLYYFDYWGQGTTLTVSS

SEQ ID NO: 497 - protein, 107 aa, Synthetic construct
DIVMTQSQKFMSTSVGDRVSITCKASQNVRTAVAWYQQKPGQSPKALIYLASNRHTGVPDRFTGSGSGTDFTLTISNVQSEDLADYFCLQHWNYPLTFGAGTKLELK

SEQ ID NO: 498 - protein, 123 aa, Synthetic construct
RVQLQQSGAELVRPGASVTLSCKASGYTFTDYEMHWVKQTPVHGLEWIGAIDPETGGTAYNQKFKGKAILTADKSSSTAYMELRSLTSEDSAVYYCTRWITTVVATLYYFDYWGQGTTLTVSS

SEQ ID NO: 499 - protein, 119 aa, Synthetic construct
EVQLQQSGPELVKPGASVKISCKASGYTFTDYYMSWVKQSHGKSLEWIGDVNPNNGDTSYNQKFKGKATLTVDKSSSTAYMELRSLTSEDSAVYYCAASGLPYVLMDYWGQGTSVTVSS

SEQ ID NO: 500 - protein, 107 aa, Synthetic construct
DIQMTQSPASLSASVGETVTITCRASENINSYLAWYQQKQGKSPQLLVYNTKTLTEDVPSRFSGSGSGTQFSLKINSLQPEDFGSYYCQHHYGTPLTFGGGTKLELK

SEQ ID NO: 501 - protein, 119 aa, Synthetic construct
EVQLVESGGGLVKPGGSLKLSCAASGFTFSGYALSWVRQTPEKRLEWVATIRDGGSYTYYSDNEKGRFTISRDNAKNNLYLQMSHLKSEDTAIYYCTRDQVNRGWFTYWGQGTLVTVSA

SEQ ID NO: 502 - protein, 119 aa, Synthetic construct
EVQLVESGGGLVKPGGSLKLSCAASGFTFSDYALSWVRQTPEKRLEWVATIRDGGSYTYYSDNEKGRFTISRDNAKNNLYLQMSHLRSEDTAMYYCTRDQVNRGWFTYWGQGTLVTVSA

SEQ ID NO: 503 - protein, 108 aa, Synthetic construct
QVILTQSPAIMSASLGERVTMTCSASSSVSSSYFHWFQQKPGSSPKLWIYSTSNLASGVPPRFSGSGSGTSYSLTISSMEAEDAATYYCHQHHRSPLTFGAGTKLELK

SEQ ID NO: 504 - protein, 120 aa, Synthetic construct
EVQLQQSGPVLVKPGASVKMSCKASGYIFTDYYMHWVKQSHGKSLEWIGIINPYNGDTSYNQKFKDKATLTVDKSSSTAYMELNSLTSEDSAVYYCARDSSNVGNAMDYWGQGTSVTVSS

SEQ ID NO: 505 - protein, 107 aa, Synthetic construct
DIQMTQTTSSLSASLGDRVTISCRASQDISNYLNWYLQKPDGTIKLLIYYSSRLHSGVPSRFSGSGSGTDYSLTISNLEQEDIATYFCQQGYTLPRTFGGGTKLEII

SEQ ID NO: 506 - protein, 107 aa, Synthetic construct
DIQMTQTTSSLSASLGDRVTISCRASQDISNYLNWYLRKPDGTVKLLIYYSSRLHSGVPSRFSGSGSGTDYSLTISNLEQEDIATYFCQQGNTLPRTFGGGTKLEIK

SEQ ID NO: 507 - protein, 119 aa, Synthetic construct
EVQLVESGGGLVKPGGSLKLSCAASGFTFSGYALSWVRQTPEKRLEWVATIRDGGSYTYYSDNEKGRFTISRDNAKNNLYLQMSHLKSEDTAMYYCTRDQVNRGWFTYWGQGTLVTVSA

SEQ ID NO: 508 - protein, 115 aa, Synthetic construct
DVQLQESGPGLVKPSQSLSLTCSVTGYSITSNYYWNWIRQFPGNNLEWMGYISSDGTNNYNPSLRNRISITRDTSKNQFFLKLNSVTTEDTATYYCARGLRYGPWGQGTTLTVSS

SEQ ID NO: 509 - protein, 111 aa, Synthetic construct
QLILTQSSSASFSLGASAKLTCTLSSQHSTYTIEWYQQQPLKAPKYVMEVKNDGSHRTGDGIPDRFSGSSSGADRYLSISNIQPEDEAIYICGVGDINNYIFGGGTKVTVL

SEQ ID NO: 510 - protein, 120 aa, Synthetic construct
EVMLVESGGGLVKPGGSLKLSCAASGFSFSSYSMSWVRQTPEKRLECVATIGGVGGNTYYPDSVKGRFSISRDNAKNTLYLQMSSLRSEDTALYYCARHEDYYYYAMDYWGQGTSVTVSS

SEQ ID NO: 511 - protein, 106 aa, Synthetic construct
QIVLTQSPAIMSASPGEKVTMTCSANSTVSYIYWYQQKPGSSPRLLIYDTSNLASGVPVRFSGSGSGTSYYLTISRMEAEDAATYYCQQWSSFPFTFGSGTKLEIK

SEQ ID NO: 512 - protein, 120 aa, Synthetic construct
EVMLVESGGGLVKPGGSLKLSCAASGFIFSSYIMSWVRQTPEKRLEWVATIRGGGGNTYYLDSVKGRFIISRDNAKNNLYLQMSSLRSEDTALYYCARHEDYEWYAMDNWGQGTSVTVSS

SEQ ID NO: 513 - protein, 106 aa, Synthetic construct
QIVLTQSPAIMSASPGEKVTLTCSARSSVSYMYWYQQKPGSSPKLLIYDTSNLASGVPVRFSGSGSGTSYSLTISRMEAEDAATYYCQQWSSYPLTFGAGTKLELK

SEQ ID NO: 514 - protein, 120 aa, Synthetic construct
EVMLVESGGDLVKPGGSLKLSCAASGFTFSSYFMSWVRQTPEKRLEWVATISGGGDKTYYLDILKGRFTISRDNAKNTLYLQMSSLRSEDTALYYCARHEDYAWYAMDYWGQGTSVTVSS

SEQ ID NO: 515 - protein, 106 aa, Synthetic construct
QIVLTQSPAIMSASPGEKVTMTCSASSSVNYIYWYQQKPGSSPRLLIYDTSNLASGVPVRFSGSGSGTSYSLTISRMEAEDAATYYCQQWSSYPLTFGAGTKLELK

SEQ ID NO: 516 - protein, 106 aa, Synthetic construct
DIQMTQSPSSLSASLGGKVTITCKASQDINKYIAWYQHKPGKGPRLLIHYTSTLQPGIPSRFSGSGSGRDYSFNISNLEPEDIATYYCLQYDNLYMFGGGTKLEIK

SEQ ID NO: 517 - protein, 119 aa, Synthetic construct
EAQLQQSGPELVKPGASVKISCKASGYTFTDYYMNWVKQSHGKSLDWIGDINPDNGGSTYNQKFKGKATLTVDKSSSTAYMELRSLTSEDSAVYYCSASGPPYVLLDYWGQGTSVIVSS

SEQ ID NO: 518 - protein, 107 aa, Synthetic construct
DIQMTQSPASLSASVGETVTITCQTSENIYSYLAWYQQKQGKSPQLLVYNTQTLAEGVPSRFSGSRSGAQFSLKINSLQPEDFGSYYCQHHYGVPLTFGAGTKLELK

SEQ ID NO: 519 - protein, 120 aa, Synthetic construct
EVQLQQSGPVLVKPGASVKMSCKASGYRLTDYYMHWVKQSHGKSLEWIGIINPYNGGTSYNQKFKGKATLTVDKSSSTAYMELNSLTSDDSAVYYCARDSSNVGNDMDYWGQGTSVSVSS

SEQ ID NO: 520 - protein, 107 aa, Synthetic construct
DIQMTQTTSSLSASLGDRVTISCRASQDISNYLNWYLQKPDGTVKLLIYYSSRLHSGVPSRFSGSGSGTDYSLTINNLEQEDIATYFCQQGNTLPRTFGGGTKLEIR

SEQ ID NO: 521 - protein, 120 aa, Synthetic construct
EVILVESGGGLVKPGGSRKLSCAASGFTFSSYFMSWVRQTPEKRLEWVATISGGGDNTYYPDSVKGRFTISRDNAKNTLYLQMSSLRSEDTALYYCARHEDYEWYAMDYWGQGTSVTVSS

SEQ ID NO: 522 - protein, 106 aa, Synthetic construct
QIVLTQSPAIMSTSPGEKVTMTCSASSSVSYIYWYQQKPGSSPRLLIYDTSNLASGVPVRFSGSGSGTSYSLTISRMEAEDAATYYCQQWTSYPLTFGAGTKLELK

SEQ ID NO: 523 - protein, 120 aa, Synthetic construct
EVQLVESGGDLVKPGGSLKLSCAASGFTFSSYFMSWVRQTPDKRLEWVATIRGGGSYTYYLDSVKGRFTVSRDNAKNTLYLQMSSLKSEDTAMYYCARHEDYDYYAMDYWGQGTSVTVSS

SEQ ID NO: 524 - protein, 106 aa, Synthetic construct
QIVLTQSPAIMSASPGEKVTMTCSASSSVSYMYWYQQKPGSSPRLLIYDTSNLASGVPVRFSGSGSGTSYSLTISRMEAEDAATYYCQQWSSYPLTFGAGTKLELK

SEQ ID NO: 525 - protein, 114 aa, Synthetic construct
QAQLQQPGAELVKPGASVKMSCKASGYTFTSYWITWVKQRPGQGLEWIGDIYPGNFSPNYNEKFKNKATLTVDTSSSTAYMQLSSLTSEDSAVYYCAKGYFDVWGTGTTVTVSS

SEQ ID NO: 526 - protein, 120 aa, Synthetic construct
EVQLQQSGPELVKPGASVKISCKASGYTFTHYYKNWVKQSHGKSLEWIGAINPNIGGPSYNQKFKGKATLTVDKSSSTVYMELRSLTSEDSAVYYCARSDDYGGYYFDYWGQGTTLTVSS

SEQ ID NO: 527 - protein, 106 aa, Synthetic construct
QIVLSQSPALLSASPGEKVTMTCRANSSVNYMHWYQQKPGSSPKPWIYATSNLASGVPARFSGSGSGTSFSLTISRVEAEDAATYYCQQWTSNPLTFGAGTKLELK

SEQ ID NO: 528 - protein, 117 aa, Synthetic construct
EVQLQQSGPELVKPGASVKISCKASGYTFTDYYMNWVRQSHGKSLEWIGDIYPNNGDTNYNQKFKGKATLTVDKSSKTADMELRSLTSEDSAVYYCIRGVGLGFPYWGQGTLVTVSA

SEQ ID NO: 529 - protein, 107 aa, Synthetic construct
DIVMTQSHKFISTSVGDGVSITCQASQVVSTAVAWYQQKPGQSPRLLLHSASFRYSGVPDRFTGSGSGTDFTFTISTVQAEDLAVYYCQQHYRTPYTFGGGTKLEIK

SEQ ID NO: 530 - protein, 120 aa, Synthetic construct
EVQLQQSGPVLVKPGASVKMSCEPSGYTFTHYYVNWMRQSHGKSLEWIGVIKPYNGAPSYNQKFKGKATLTVDKSSSKINMELNSLTSEDSAVYYCARSDDFDGYAMDYWGQGTSVTVSS

SEQ ID NO: 531 - protein, 106 aa, Synthetic construct
QIVLTQSPAIMFASPGEKVTMTCSASSSVSYMHWYQQKSGTSPKRCISDTSKLASGVPARFSGSGSGTSYSLTISSMEAEDAATYYCQQWTSNPLTFGSGTKLELK

SEQ ID NO: 532 - protein, 120 aa, Synthetic construct
EVQLVESGGDLVKPGGSLKLSCAASGFTFNNYGMSWVRQTPDKRLEWVATISRGGSFTYYPDSVKGRFTISRDNAKNTLYLQMSSLKSEDTAMYYCARPIYYEYDGFAYWGQGTLVTVSA

SEQ ID NO: 533 - protein, 112 aa, Synthetic construct
DVLMTQTPLSLPVSLGDQASISCRSSQSIVHSNGNTYLEWYLQKPGQSPKLLIYKVSNRFSGVPDRFSGSGSGTDFTLKINRVEAEDLGVYSCFQGSHVPRTFGGGTKLEIK

SEQ ID NO: 534 - protein, 114 aa, Synthetic construct
QVQLQQPGAELVKAGASVKMSCKASGYTFTSYWITWVKQRPGQGLEWIGDIYPGNDSPNYNEKFKNKATLTVDTSSSTAYMQLSSLTSEDSALYYCARGYYDYWGQGTTLTVSS

SEQ ID NO: 535 - protein, 113 aa, Synthetic construct
DIVMTQSPSSLSVSAGEKVTMSCKSSQSLLNSGNQKNYLAWYQQKTGQPPKLLIYGASTRESGVPDRFTGSGSGTDFTLTISSVQAEDLAVYYCQNDHSYPHTFGAGTKLELK

SEQ ID NO: 536 - protein, 113 aa, Synthetic construct
EVQLQQSGPVLVKPGASVKMSCKASGNTFNGYYVNWVKQSHGKSLEWIGLIDPSNGGTNYNQKFKDKATLTVDKSSTTAYMEFNSLTSEDSSVYYCAGGTVYWGQGTTLTVSS

SEQ ID NO: 537 - protein, 107 aa, Synthetic construct
DIQMTQSPSSLSASLGERVSLTCRASQDIGNNLNWLQQEPDGTIKRLIYATSSLDSGVPKRFSGSRSGSDYSLTISSLESEDFVDYYCLQYASSPVTFGGGTKLEIK

SEQ ID NO: 538 - protein, 120 aa, Synthetic construct
EVQLQQSGPELVKPGASVKISCKASGYMFTDYYMNWVKQSHGGSLEWIGTFNPNRGGPSYNLKFKGKATLTVDKSSITAYMDLRSLTSEDSAVYYCARADDYDGYYFDYWGQGTTLTVSS

SEQ ID NO: 539 - protein, 106 aa, Synthetic construct
QIVLTQSPAIMSASPGEKVTMTCSASSSVSYMHWYQQKSGTSPKRWIYDTSKLASGVPARFSGSGSGTSYSLTISSMEAEDAATYYCQQWTNNPLTFGAGTKLELK

SEQ ID NO: 540 - protein, 115 aa, Synthetic construct
QVQLQQSGPELVKPGASVRISCKASGYSFTDYFISWVKQRPGQGLEWIGWIFPGSGSTYFNENFKGEATLTADKSSSTAYLLLSSLTSEDSAVYFCTTYYGSNYWGQGTTLTVSS

SEQ ID NO: 541 - protein, 112 aa, Synthetic construct
DVLMTQAPLSLPVSLGDQASISCRSSQSIVHSNGNTYLEWYLQKPGQSPKLLIYTVSNRLSGVPDRFSGSGSGTDFTLKISRVEAEDLGIYYCFQTSHVPPTFGGGTKLEIK

SEQ ID NO: 542 - protein, 106 aa, Synthetic construct
DIQMTQSPSTLSASVGDRVTITCRASQSISSWLAWYQQKPGKAPKVLIYKASTLESGVPSRFSGSGSGTDFTLTISSLQPEDFATYNCQQYNTYWTFGQGTKVEIK

SEQ ID NO: 543 - protein, 114 aa, Synthetic construct
EVQLQQSGPELVKPGASVKISCKASGYTFTDYSMNWVKQSHGKSLEWIGDINPNNGGTSYNQKFKGKATLTVDKSSSTAYMELRSLTSEDSAVYYCARVWFAYWGQGTLVTVSA

SEQ ID NO: 544 - protein, 113 aa, Synthetic construct
DIVMTQSPSSLSVSAGEKVTLSCKSSQSLLNSGNQKNYLAWYQQKPGQPPKLLIYGASTRESGVPDRFTGSGSGTDFTLTISSVQAEDLALYYCQNAHSYPFTFGSGTKLDIK

SEQ ID NO: 545 - protein, 118 aa, Synthetic construct
QHELQQSGAELVRPGSSVKLSCKDSYFAFMASAMHWVKQRPGHGLEWIGSFTMYSDATEYSENFKGKATLTANTSSNTAYMELSSLISEDSAVYYCASGYSGNGFTYWGQGTLVTVSA

SEQ ID NO: 546 - protein, 112 aa, Synthetic construct
DIVLTQSPASLAMSLGQRATISCRASESVDNYGISFMHWYQQKPGQPPKLLIYRASNLESGIPARFSGSGSRTDFTLTINPVETDDVATYYCQQSNKDPMYTFGGGTKLEIR

SEQ ID NO: 547 - protein, 114 aa, Synthetic construct
QVQLQQPGAELVKPGASVNMSCKASGYTFSSYWITWVKQRPGQGLEWIGDIHPGNTSPNYNEKFRTKATLTVDTSSSTAYMQLSSLTSEDSAVYYCARGWGDYWGQGTTLTVSS

SEQ ID NO: 548 - protein, 113 aa, Synthetic construct
DIVMTQSPSSLSVAAGEKVTMSCKSSQSLLNSGNQKNYLAWYQQKPGQPPKLLIYGASTRESGVPDRFTGSGSGTDFTLTISSVQAEDLAVYYCQNDHGYPLTFGTGTKLELK

SEQ ID NO: 549 - protein, 121 aa, Synthetic construct
EVQLVESGGDLVKPGGSLKLSCVASGLTFSDYGMYWIRQAPEKGLEWVAYIRSDSSTIYYTDTVKGRFTISRDNAKNTLFLQMTSLRSEDTAIYYCARRSPVVVNYAMDYWGQGTSVTVSS

SEQ ID NO: 550 - protein, 107 aa, Synthetic construct
DIQMTQSPASLSASVGETVTITCRASENIYSHLVWYQQKQGKSPHLLVYNGKILAEGVPSRFSGSGSGTQFSLKINSLQPEDFGSYYCQHHYGSPITFGAGTKLELN

SEQ ID NO: 551 - protein, 120 aa, Synthetic construct
EVQLQQSGPELVKPGTSVKISCKASGYTFTDYYMNWVRQSHGKSLEWIGEINPKNGDTNYNQNFKGKATLTVDKSSNTAYMELRSLTSEDSAVFYCAREGVSSYYAMDYWGQGTSVTVSS

SEQ ID NO: 552 - protein, 113 aa, Synthetic construct
DIVMTQSPSSLAMSVGQKVTMSCKSSQSLLNSFNQKNFLAWYQQKPGQSPKLLVYFASTRESGVPDRFIGSGSGTDFTLTITSVQAEDLADYFCQQHHSTPPTFGGGTKLEIN

SEQ ID NO: 553 - protein, 113 aa, Synthetic construct
EVQLQQSGPVLVKPGASVKMSCKASGNTFNGYYINWVKQSHGKSLEWIGLIDPSNGGTNYNQKFKDKATLTVDKSSTTAYMEFNTLTSEDSSVYYCAGGTVYWGQGTTLTVSS

SEQ ID NO: 554 - protein, 107 aa, Synthetic construct
DIQMTQSPSSLSASLGERVSLTCRASQDIGNNLNWLQQEPDGTIKRLIYATSSLDSGVPKRFSGSRSGSDYSLTISSLESEDFVDYYCLQYASSPPTFGGGTKLEIK

SEQ ID NO: 555 - protein, 121 aa, Synthetic construct
EVQLVESGGGLVKPGGSLKLSCAASGITFSDYGMHWVRQAPEKGLEWVAYIRSDSSTIYYADTVKGRFTISRDNAKNTLFLQMTSLRSDDTAMYYCARRSPVVVNYAMDYWGQGTSVTVSS

SEQ ID NO: 556 - protein, 107 aa, Synthetic construct
DIQMTQSPASLSASVGETVTITCRASENIYSYLVWYQQKQGKSPQLLVYNGKILAEGVPSRFSGSGSGTQFSLKINSLQPEDFGSYYCQHHYGSPLTFGAGTKLELK

SEQ ID NO: 557 - protein, 120 aa, Synthetic construct
EVHLQQSGPELVKPGASVKISCKASGYTFTDYYMNWMKQSHGKGLEWIGEINPKNGDTNYSQKFRDKATLTVDKSSNTAFMKLRSLTSEDSAVYFCAKEGVGSYYAMDYWGQGTSVTVSS

SEQ ID NO: 558 - protein, 113 aa, Synthetic construct
DIVMTQSPSSLAMSVGQKVTMSCKSSQSLLSSNNQKSFLAWYQQKPGQSPKLLVSFASTRESGVPDRFIGGGSGTDFTLTISSVQPEDLADYFCQQHYSTPPTFGEGTKLEIK

SEQ ID NO: 559 - protein, 114 aa, Synthetic construct
QVQLQQPGAELVKAGASVKMSCKASGYTFTSYWITWVKQRPGQGLEWIGDIYPGNDSPNYNEKFKNKATLTVDTSSSTAYMQLSSLTSEDSAVYYCTRGYYDYWGQGTTLTVSS

SEQ ID NO: 560 - protein, 113 aa, Synthetic construct
DIVMTQSPSSLSVSAGEKVTMSCKSSQSLLNSGNQKNYLAWYQQKPGQPPKLLIYGASTRESGVPDRFTGSGSGTDFTLTISSVQAEDLAVYYCQNDHSYPHTFGAGTKLELR

SEQ ID NO: 561 - protein, 113 aa, Synthetic construct
EVQLQQSGPVLVKPGASVKMSCKASGNTFNGYYINWVKQRHGKSLEWIGLIDPSNGGTNYNQKFKDKATLTVDKSSTTAYMEFNSLTSDDSSVYYCAGGTVYWGQGTTLTVSS

SEQ ID NO: 562 - protein, 120 aa, Synthetic construct
EVQLQQSGPELVKPGASVKISCKASGYMFTDYYMNWVKQSHGKSLEWIGEINPNNGDTNYSQKFRDKATLTVDKSSNIAFMELRSLTSEDSAVYFCAKEGVSSYYAMDYWGQGTSVTVSS

SEQ ID NO: 563 - protein, 113 aa, Synthetic construct
DIVMTQSPSSLAMSVGQKVTMSCKSSQSLLNSNNQKNFLAWYQQKPGQSPKLLVYFASTRESGVPDRFIGGGSGTDFTLTISNVQPEDLADYFCQQHYSTPPTFGGGTKLEIK

SEQ ID NO: 564 - protein, 120 aa, Synthetic construct
EVQLQQSGPELVKPGTSVKISCKASGYTFTDYYMNWVRQSHEKSLEWIGEINPKNGDTNYNQNFKAKATLTVDKSSNTAYMELRSLTSEDSAVFYCAREGVSSYYGMDSWGQGTSVTVSS

SEQ ID NO: 565 - protein, 113 aa, Synthetic construct
DIVMTQSPSSLAVSVGQKVTMSCKSSQSLLNGFNQKNFLAWYQQKPGQSPKLLVYFASTRESGVPDRFIGSGSGTDFTLTITSVQAEDLADYFCQQHHSTPPTFGGGTKLEIN

SEQ ID NO: 566 - protein, 114 aa, Synthetic construct
EVQLQQSGPELVKPGASVKMSCKASGYTFTDYSMNWVKQSHGKSLEWIGDINPNNGGTNYNQKFKGKATLTVDRSSSTAYMELRSLTSEDSAVYYCARVWFAYWGQGTLVTVSA

SEQ ID NO: 567 - protein, 113 aa, Synthetic construct
DIVMTQSPSSLSVSEGEKVTMSCKSSQSLLSSGNQKNFLAWYQQKAGQPPKLLIYGASTRESGVPDRFTGSGSGTDFTLTISSVQAEDLAVYYCQNAHSSPFTFGSGTKLEIK

SEQ ID NO: 568 - protein, 114 aa, Synthetic construct
EVQLQQSGPELVKPGASVKISCKASGYTFTDYSMNWVKQSHGKSLEWIGDINPDNGGTSYNQKFKGKATLTVDQSSSTAYMELRSLTSEDSAVYYCARIWFAYWGQGTLVTVSA

SEQ ID NO: 569 - protein, 113 aa, Synthetic construct
DIVMTQSPSSLSVSAGEKVTMSCKSSQSLLNSGIQKNFLAWYQQKPGQPPKLLIYGASTRESGVPDRFTGSGSGTDFTLTISSVQAEDLAVYYCQNAHSYPFTFGSGTKLEIK

SEQ ID NO: 570 - protein, 120 aa, Synthetic construct
EVQLQQSGPELVKPGASVKISCKASGYTFTDYYMNWVRQSHEKSLEWIGEINPNNGDTNFNQKFKGKATLTVDKSSSTAFMDLRSLTSKDSAVYYCAREGGSSYYAMDYWGQGTSVTVSS

SEQ ID NO: 571 - protein, 113 aa, Synthetic construct
DIVMTQSPSSLAMSVGQKVTMSCKSSQSLLSNNNQKNFLAWYQQKPGQSPKLLVYFASTRESGVPDRFIGSGSGTDFTLTISSVQAEDLADYFCQQHYSTPPTFGGGTKVEIK

SEQ ID NO: 572 - protein, 119 aa, Synthetic construct
EVQLQQSGPELVKPGSSVKISCEASGFTFADYNVDWVKQSHGKSLEWIGAINPNDGGTSYNQKFEGKATLTVDKSSTTAYMELRSLTSEDSAVYYCARWVNNDWYFDVWGTGTTVTVSS

SEQ ID NO: 573 - protein, 107 aa, Synthetic construct
DIVMTQSQKFMSTSVGDRVSITCKASQNVRSAVDWYQQKPGQSPKTLIHSASNRHTGVPDRFTGSGSGTDFTLTISNIQSEDLADYFCLQHWNYPYTFGGGTKLEVK

SEQ ID NO: 574 - protein, 119 aa, Synthetic construct
QVQLQQSGAELARPGASVKLSCKASGYTFTNYGISWVKQRTGQGLEWIGEIYPGTINIYYSERFKGKATLTADKSSSTAYMQLTSLTSEDSAVYFCARDDGYYDAMDYWGQGTSVTVSS

SEQ ID NO: 575 - protein, 107 aa, Synthetic construct
DIQMTQSPSSLSASLGQKVILTCRASQDIGSSLNWLQQEPDGTIKRLIYATSSLDSGVPKRFSGSRSGSDYSLTISSLESEDFVVYYCLQYTSSPWTFGGGTKLEIK

SEQ ID NO: 576 - protein, 123 aa, Synthetic construct
QVQLQQPGAELVKPGASVKLSCKASGYTFTSYWMHWVKQRPGQGLEWIGEIDPSDSYTNYNQKFKGKATLTVDKSSSTAYMQLSSLTSEDSAVYYCASSIYYSNYVRYYFDYWGQGTTLTVSS

SEQ ID NO: 577 - protein, 119 aa, Synthetic construct
EVQLQQSGPELVKPGSSVKISCEASGYTFADYNVDWVKQSHGKSLEWIGAINPNDGGTSYNQKFEGKATLTVDKSSTTAYMELRSLTSEDSAVYYCARWVINDWYFDVWGTGTTVTVSS

SEQ ID NO: 578 - protein, 106 aa, Synthetic construct
DIQMTQSPSSLSASLGGKVTITCKASQDINKYIAWYQHKPGKGPRLLIHYTSTLQPGIPSRFSGSGSGRDYSFSISNLEPEDIATYYCLQYDNLWTFGGGTKLEIK

SEQ ID NO: 579 - protein, 119 aa, Synthetic construct
EVQLQQSGPELVRPGSSVKISCKASGYTFTDYNMDWVKQSHGKSLEWIGANDPKNGGFSYNQRFKGKATLTVDKSSSTAYMELRSLTSEDSAVYYCARWDSNYWYFDVWGTGTTVTVSS

SEQ ID NO: 580 - protein, 107 aa, Synthetic construct
DIVMTQSQKFMSTSIGDRVSITYKASQDVRSAVAWYQQKPGQSPKALIYLASNRHTGVPDRFTGSGSGTDFTLTITNVQSEDLADYFCLQHWTYPYTFGGGTKLEIK

SEQ ID NO: 581 - protein, 119 aa, Synthetic construct
EVQLQQSGPELVKPGSSMKISCKASGYTFTDYSMDWVKQSHGKSLEWIGAINPNNGGTSYNQKFKDKATLTVDRSSSTAYMELRSLTSEDSAVYYCARWDSDYWYFDVWATGTTVTVSS

SEQ ID NO: 582 - protein, 107 aa, Synthetic construct
DIVMTQSQKFMSTSVGDRVSITCKASQNVRTAVDWYQQKPGQSPKALIYSASNRHTGVPDRFTGSGSGTDFTLTISNVQSEDLADYFCLQHWNYPYTFGGGTKLEIK

SEQ ID NO: 583 - protein, 118 aa, Synthetic construct
EVQLQQSGPELVKPGSSVKISCKASGYTFTDYNMDWVKQSHGQSLEYIGAVNPNTGDISYTQKFKDKATLTVDKSSSTAYMELRSLTSEDSAVYYCARWSESWYFDVWGTGTTVTVSS

SEQ ID NO: 584 - protein, 107 aa, Synthetic construct
DIVMTQSQKLMSTSVGDRVSITCKASQNVRAAVDWYQQKPRQSPKALIFLASSRHTGVPDRFTGSGSGTDFTLTITNVQSEDLATYFCLQHWNYPYTFGGGTRVEIK

SEQ ID NO: 585 - protein, 119 aa, Synthetic construct
EVQLQQSGPELVKPGSSVKISCKASGYTFTDYNIDWVKQSHGKSLEWIGAIDPNNGGTNYNQKFKDKATLTVDKSSSTAYMELRSLTSEDSAVYYCTRWDSNDWYFDVWATGTTVTVSS

SEQ ID NO: 586 - protein, 107 aa, Synthetic construct
DIVMTQSQKFMSTSVGDRVSITCKASQNVRIAVDWYQQKPGQSPKALIFSSSNRHTGVPDRFTGSGSGSDFTLTIRNVQSEDLADYFCLQHWISPYTFGGGTKLEIR

SEQ ID NO: 587 - protein, 119 aa, Synthetic construct
EVQLQQSGPELAKPGSSVKISCKASGYTFTDYNIDWVKQSHGKSLEWIGAIDPNNDSTNYNQKFKGKATLTVDKSSSTAYMELRSLTSEDSAVYYCTRWDSDDWYFDVWATGTTVTVSS

SEQ ID NO: 588 - protein, 107 aa, Synthetic construct
DIVMTQSQKFMSTSVGDRVSITCKASQNVRSAVDWYQQKPGQSPKALIFSSSNRHTGVPDRFTGSGSGTDFTLTIRNVQSEDLADYFCLQHWNSPYTFGGGTKLEIR

SEQ ID NO: 589 - protein, 107 aa, Synthetic construct
DIQMTQSSSSFSVSRGDRVTITCKASEDIYNRLAWYQQKPGNAPRLLISGTTSLEIGFPSRFSGSGSGKDYTLSISSLQTEDVATYYCQQYWSTPWTFGGGTKLEIK

SEQ ID NO: 590 - protein, 123 aa, Synthetic construct
EVQLQQSGAELAKPGASVKLSCTVSGFNIKDTYIHWVKQRPEQGLEWIGGIDPAIGNTVSASKFQDKATITADTSSSTAYMQLSSLTSGDTAVYYCARERVHSNTLYYAMDYWGQGTSVTVSS

SEQ ID NO: 591 - protein, 111 aa, Synthetic construct
DIVLTQSPASLAVSLGQRATISCRASKSVSISGYSYMHWYQQKPGQPPKLLIYLASNLESGVPARFSGSGSGTDFTLNIHPVEEEDAATYYCQHSRELPPTFGGGTKLEIK

SEQ ID NO: 592 - protein, 120 aa, Synthetic construct
QVQLQQSGPELARPGASVKLSCKASGYTLTSHGISWVKQRTGQGLEWIGEIYPGSESPYYSEKFKGKATLTADKSSNIAYMQLSSLTSEDSAVYFCARSDYSDYWAMDYWGQGTSVTVSS

SEQ ID NO: 593 - protein, 107 aa, Synthetic construct
DIVMTQSQKCMSTSVGDRVSITCKASQNVRSAVAWYQQKPGQSPKTLIYLASNRHTGVPDRFTGSGSGTDFTLTITNVQSEDLADYFCLQHWNYPWTFGGGTELEIK

SEQ ID NO: 594 - protein, 107 aa, Synthetic construct
EIVMTQSPATLSVSPGERATLSCRASQSVSSNLAWYQQKPGQAPRLLIYGASTRATGIPARFSGSGSGTEFTLTISSLQSEDFAVYYCHQYNNWPRTFGQGTKVEIK

SEQ ID NO: 595 - protein, 120 aa, Synthetic construct
QVQLQQPGAELVKPGASVKLSCKASGYTFTSSWMHWVKQRPGQGLEWIGEINPSDGRTNYNEKFKSKATLTVDHSSSTAYMQLSSLTSEDSAVYYCASNADRAYYTMDYWGQGTSVTVSS

SEQ ID NO: 596 - protein, 113 aa, Synthetic construct
DIVMTQSPSSLAMSVGQKVTMSCKSSQSLLNSFNQRNFLAWYQQKPGQSPKLLVYFASTRDSGVPDRFIGSGSGTDFTLTISSVQAEDLADYFCQQHYSTPPTFGGGTKLEIK

SEQ ID NO: 597 - protein, 119 aa, Synthetic construct
EVQLQQSGPELVKPGSSVKISCKASGYTFTDYNLDWMKQSHGSSLEWIGAMSPNNGATSYNQKFKGKATLTVDKSSSTAYMELRSLTSEDSAVYYCARWDSNSWYFDVWGTGTTVTVSS

SEQ ID NO: 598 - protein, 107 aa, Synthetic construct
DIVMTQSQKFMSTSVGDRVSITCKASQIVRTAVDWYQQKSGQSPKALIYSASTRHTGVPDRFTGSGSGTDFTLTIDNVQSEDLAEYFCLQHWNYPYTFGGGTKLEIK

SEQ ID NO: 599 - protein, 114 aa, Synthetic construct
QVQLQQSGAELVRPGTSVKMSCKAAGYTFTNSWINWVKQRPGHGLEWIGDIYPGNTFPNYNEKFKGKATLTADTSSSTAYMQLSSLTSEDSAVYYCTGGYFDVWGTGTTVTVSS

SEQ ID NO: 600 - protein, 113 aa, Synthetic construct
DIVMTQSPSSLSVSAGEKVTMSCKSSQSLLNSGNQKNFLAWYQQKPGQPPKLLIFGASTRQSGVPDRFTGSGSGTDFTLTISSVQAEDLAVYYCQNDHSYPYTFGGGTKLEMK

SEQ ID NO: 601 - protein, 123 aa, Synthetic construct
EVQLQQSGAELVKPGASVKLSCTASGFNIEDTYIHWVKRRPEQGLEWIGGIDPAIGNTLYASKFQDMATITADTSSSTAYMQLSSLTSGDTAVYYCARERVYSNTLYYAMDYWGQGTSVTVSS

SEQ ID NO: 602 - protein, 111 aa, Synthetic construct
DIVLTQSPASLVVSLGQRATISCRASKSVSISGYSYMHWYQQKPGQPPKLLIYLASNLESGVPARFSGSGSGTDFTLNIHPVEAEDAATYYCQHSRELPPTFGGGTNLEIK

SEQ ID NO: 603 - protein, 119 aa, Synthetic construct
EVKLVESGGGLVQPGGSLKLSCAVSGFTFSSYTMSWVRQTPEKRLELVAKISNSGGSTNYPDTVKGRFTLSRDNVKNTLYLQMSSLKSEDTAIYYCTRYSWDVYAMDYWGQGTSVTVSS

SEQ ID NO: 604 - protein, 106 aa, Synthetic construct
DIQMTQSPASLSASVGETVIITCRASENIYSYLAWYQQKQGKSPHLLVYNAETLVEGVPSRFSGSGSATQFSLKINSLQPEDFGTYYCQHHYGDPTFGGGTKLEIK

SEQ ID NO: 605 - protein, 116 aa, Synthetic construct
QVQLQQSGAELARPGASVKMSCKASGYTFTDYWMQWVKQRPGQGLEWIGAIFPGNGETRDTQKFKGRATLTADRSSSTAYIQLSSLTSEDSAVYYCATFNNYLDYWGQGTTLTVAS

SEQ ID NO: 606 - protein, 106 aa, Synthetic construct
QIVLTQSPAIMSASPGEKVTMTCSASSSVSYMHWYQQKSGASPKRWIYDTSKLTSGVPARFSGSGSGTSYSLTISNMEAEDAATYYCQQWISNPYTFGGGTKLEIK

SEQ ID NO: 607 - protein, 120 aa, Synthetic construct
QVQLQQPGAELVKPGTSVKLSCKAAGYIFTSSWMHWVKQRPGQGLEWIGEINPSDGRTNYNEKFKNKATLTVDHSSSTAYMQLSSLTSEDSAVYYCASNADRAYYTMDYWGQGTSVTVSS

SEQ ID NO: 608 - protein, 113 aa, Synthetic construct
DIVMTQSPSSLAMSVGQKVTMSCKSSQSLLNGFNQRNFLAWYQQKPGQSPKLLVYFASTRDSGVPDRFIGSGSGTDFTLTISSVQAEDLADYFCQQHYSTPPTFGGGTKLEIK

SEQ ID NO: 609 - protein, 118 aa, Synthetic construct
EVKLVESGGGLVQPGGSLKLSCVASGFTFNTYIMSWVRQTPEKRLELVADISNSGGNTYYSDTVKGRFTISRDNAKNTLYLQMSSLKSEDTAMYYCARPDNWDPFVYWGQGTLVTVSA

SEQ ID NO: 610 - protein, 107 aa, Synthetic construct
DIQMTQSSSSFSVSLGDRVTITCKASEDIYARLAWYQQKPGNAPRLLISGATSLETGVPSRFSGSGSGKNYTLSITSLQTEDVGTYYCQQHWSTPWTFGGGTNLEIK

SEQ ID NO: 611 - protein, 114 aa, Synthetic construct
EVQLQQSGPEVVKPGASVKISCKASGNTLTDYFINWVKQSHGKNLEWIGDINPDNGAGNYNQKFKGKATLTVDKSSGTAFMGLRSLTSEDSAVYYCATLYFDYWGQGTTLTVSS

SEQ ID NO: 612 - protein, 113 aa, Synthetic construct
DIVMTQSPSSLSVSTGEKVTMSCRSSQSLLNSGNQKNYLAWYQQKPGQPPKLLIYGASTRESGVPDRFTGSGSGTDFTLTISSVQAEDLAIYYCQNAHTSPYTFGGGTRLEIK

SEQ ID NO: 613 - protein, 114 aa, Synthetic construct
EVQLQQSGPEVVKPGASVKISCKASGNTFTDYFINWVKQSHGKSLEWIGDINPDNGGTNYNQKFKGKATLTVDKSSGTAFMGLRSLTSEDSAVYYCATLYFDYWGQGTSLTVSS

SEQ ID NO: 614 - protein, 113 aa, Synthetic construct
DIVMTQSPSSLSVSAGEKVTMSCKSSQSLLNSGNQKNYLAWYQQKPGQPPKLLIYGASTRESGVPDRFTGSGSGTDFTLTISSVQAEDLAVYYCQNAHSSPYTFGGGTRLEIK

SEQ ID NO: 615 - protein, 114 aa, Synthetic construct
EVQLQQSGPEVVKPGASVKISCKASGNTFTDYFINWVKQRHGKSLEWIGDVNPDNGGTNYNQKFKGKATLTVDKSSGTAFMGLRSLTSEDSAVYYCATLFFDSWGQGTTLTVSS

SEQ ID NO: 616 - protein, 113 aa, Synthetic construct
DIVMTQSPSSLNVSAGEKVTMSCKSSQSLLNSGNQKNYLAWYQQKPGQPPKLLIYGASTRESGVPDRFTGSGSGTDFTLTISSVQAEDLALYYCQNAHSSPYTFGGGTKLEIK

SEQ ID NO: 617 - protein, 120 aa, Synthetic construct
EVQLVESGGGLVKPGGSLKLSCAASGFTFSNFAMSWVRQTPAMRLESVATIVNGGINTYYPDTVKGRFTVSRDNAKNTLYLQMSSLRSEDTAIYYCARHDDFLYYAMDYWGQGTSVTVSS

SEQ ID NO: 618 - protein, 106 aa, Synthetic construct
QIVLTQSPAIMSASPGEKVTMTCSASSSVSYMFWYQQKPGSSPRLLIYDTSNLASGVPVRFSGSGSGTSYSLTISRLEAEDAATYYCQQWTSYPLTFGAGTKLDLK

SEQ ID NO: 619 - protein, 120 aa, Synthetic construct
EVQLVESGGGLVKPGGSLKLSCAASGFTFSSFAMSWVRQTPAKRLESVATINNGGINTYYPDTVKGRFTVSRDNAKNTLYLQMSSLRSEDTAMYYCARHDDFLYYAMDYWGQGTSVTVSS

SEQ ID NO: 620 - protein, 106 aa, Synthetic construct
QIVLTQSPAIMSASPGEKVTMTCSASSSVSYMYWYQQKPGSSPRLLIYDTSNLASGVPVRFSGSGSGTSYSLTISRMEAEDAATYYCQQWTSYPLTFGAGTKLELK

SEQ ID NO: 621 - protein, 119 aa, Synthetic construct
EVKLVESGGGLVQPGGSLKLSCAASGFTFSSYTMSWVRQTPEKRLELVAELSNSGGSFHYPDNVKGRFTISRDNAKNTLYLQMSSLKSEDTAMYYCARHNWDVYAMDYWGQGTSVTVSS

SEQ ID NO: 622 - protein, 106 aa, Synthetic construct
DIQMSQSPASLSASVGETVTITCRASENVNSYLAWYQQKQGRSPQFLVYNAQTLAEGVPSRFSGGGSGTQFSLKINSLQPEDFGSYYCQHHYGNPTFGGGTKLEIK

SEQ ID NO: 623 - protein, 120 aa, Synthetic construct
QVQLQQSGAELMTPGSSVKLSCKATGYTFTDYWIEWVKKRPGHGLEWIGEILPGYISTNYNEKFKDKATFTADTSSNTTYMQLSSLTSEDSAVYYCVLIVTTYYYFMDYWGQGTSVTVSS

SEQ ID NO: 624 - protein, 106 aa, Synthetic construct
QIVLTQSPAIMSASPGEKVTITCSASSSVTYMHWFQQKPGTSPKLWIYSTSNLASGVPVRFSGSGSGTSYSLTISRMEAEDAATYYCQQRSSYPWTFGGGTKLEIK

SEQ ID NO: 625 - protein, 120 aa, Synthetic construct
QVQLQQSGAELMKPGSSVNLSCKATDYTFTDYWINWVKQRPGHGLEWIGEILPGSVTTNYNEKFRGKATFTADTSSNTAYMQLSSLTSEDSAVYFCARGSDYSYYAMDYWGQGTSVTVSS

SEQ ID NO: 626 - protein, 113 aa, Synthetic construct
DIVMTQSPSSLAMSVGQKVTMSCKSSQSLLNIFNQKNFLAWYQQKPGQSPKLLVYFASTRESGVPDRFIGSGSGTDFTLTISNVQAEDLADYFCQQHYSTPPTFGGGTKLEIK

SEQ ID NO: 627 - protein, 118 aa, Synthetic construct
DVQLVESGGGLVKPGGSLKLSCAASGFSFSENYMYWVRQTPEKRLEWVATISDGASYTYYPDNVKGRFTISRDTAKNNLYLQMSHLKSEDTAMYYCTRDELIAPFAYWGQGTLVTVSA

SEQ ID NO: 628 - protein, 107 aa, Synthetic construct
DIVMTQSHKFMSTSVGDRVSITCKASQDVGTAVAWFQQKPGQSPKLLIYWASTRHTGVPDRFTGSGSGTDFTLTISNVQSEDLADYFCQQYNSYPWTFGGGTKLEIK

SEQ ID NO: 629 - protein, 120 aa, Synthetic construct
EVQLVESGGGLVKPGGSLKLSCAASGFTFSSYAMSWVRQTPAKRLEWVATITSGDIRTYYPDTVKGRFTISRDNAKNTLYLQMRSLRSEDTAMYYCVGHDDFHFYAMDYWGQGTSVTVSS

SEQ ID NO: 630 - protein, 106 aa, Synthetic construct
QIVLTQSPAIMSASPGEKVTMTCSASSSVSYLYWYQQKPGSSPRLLIYDTSNLASGVPVRFSGSGSGTSYSLTLSRMEAEDAATYYCQQWSSYPLTFGAGTKLELK

SEQ ID NO: 631 - protein, 120 aa, Synthetic construct
QVQLQQSGAELARPGTSVKMSCKASGYIFTNYWMNWVQQRPGQGLEWIGAINPSNGYIGYNQKFKDKATLTADKSSNTAYMQLRSLTSEDSAIYYCTRGEDFDGYAMDYWGQGTSVTVSS

SEQ ID NO: 632 - protein, 106 aa, Synthetic construct
DIQMTQSPSSLSASLGGKVTITCKASQDINKYIAWYQHKPGKGPRLLIHYTSTLQPGIPSRFSGSGSGRDYSFSISNLEPEDIATYYCLQYDNLLTFGAGTKLELK

SEQ ID NO: 633 - protein, 106 aa, Synthetic construct
QIVLTQSPAIMSASPGEKVTMTCSASSSVNYMFWYQQKPGSSPRLLIYDTSNLASGVPVRFSGSGSGTSYSLTISRLEAEDAATYYCQQWTSYPLTFGAGTKLDLK

SEQ ID NO: 634 - protein, 114 aa, Synthetic construct
EVQLQQSGPEVVKPGASVRISCKASGNTFTDFFINWVKQSHGKSLEWIGDVNPDSNGANYNQKFKGKATLTVDKSSGTAFMGLRSLTSEDSAVYYCATLFFDNWGQGTTLTVSS

SEQ ID NO: 635 - protein, 113 aa, Synthetic construct
DIVMTQSPSSLNVSAGEKVTMSCKSSQSLLNSGNQKNYLAWYQQKPGQPPKLLIYGASTRESGVPDRFTGSGSGTDFILTISSVQAEDLALYYCQNAHSSPYTFGGGTKLEIK

SEQ ID NO: 636 - protein, 119 aa, Synthetic construct
EVQLQQSGPELVKPGSSVKISCEASGYTFADYNVDWVKQSHGKSLEWIGAINPNDGGTSYNQKFEGKATLTVDKSSTTVYMELRSLTSEDSAVYYCARWVNNDWYFDVWGTGTTVTVSS

SEQ ID NO: 637 - protein, 107 aa, Synthetic construct
DIVMTQSQKFMSTSVGDRVSITCKASQNVRSAVDWYQQKPGQSPKTLIHSASSRHTGVPDRFTGSGSGTDFTLTISNIQSEDLADYFCLQHWNYPYTFGGGTKLEVK

SEQ ID NO: 638 - protein, 119 aa, Synthetic construct
EVQLQQSGPELLKPGSSVNISCKASGYTFTDYNIDWVKQSRGKSLEWIGAINPNNGGTFYNQKFKGQATLTVYKSSSTAYMELRSLTSEDSAVYYCVRWDSDSWYFDVWGTGTAVTVSS

SEQ ID NO: 639 - protein, 107 aa, Synthetic construct
DIVMTQSQKFMSTSVGERVSITCKASENVRAAVDWYQQKPGQSPKALIYLASNRHTGIPDRFTGSGSGTDFTLIISNVQSEDLADYFCLQHWNYPYTFGGGTKLEIT

SEQ ID NO: 640 - protein, 119 aa, Synthetic construct
EVQLQQSGPELAKPGSSVKISCKASGYTFTDYNIDWVKESHGKSLEWIGAIDPNNGGTNYNQKFKGKATLTVDKSSSTAYMELRSLTSEDSAVYYCTRWDSNDWYFDVWATGTTVTVSS

SEQ ID NO: 641 - protein, 107 aa, Synthetic construct
DIVMTQSQKFMSTSVGDRVSITCKASQNVRSAVDWYQQKPGQSPKALIFSSSNRHTGVPDRFAGSGSGTDFNLTIRNVQSEDLADYFCLQHWNSPYTFGGGTKLEIR

SEQ ID NO: 642 - protein, 117 aa, Synthetic construct
QVTLKESGPGILQPSQTLSLTCSFSGFSLSTFGLGIGWIRQPSGKGLEWLAHIWWDDDKYYNPALKSRLTISKDTSKNQVFLKIANVDTADTATYYCATGTYWFTYWGQGTLVTVSA

SEQ ID NO: 643 - protein, 112 aa, Synthetic construct
DVLMTQTPLSLPVSLGDQASISCRSSQSIEHSNGNTYLQWYLQKPGQSPKLLIYKVSNRFSGVPDRFSGSGSGTDFTLKISRVEAEDLGVYYCFQGSHVPWTFGGGTKLEIK

SEQ ID NO: 644 - protein, 120 aa, Synthetic construct
EVQLQQSGPVLVKPGASVKMSCKASGYRLTDYYMHWVKQSHGKSLEWIGIINPYNGDTSYNQKFKGKATLTVDKSSSTAYMELDGLTSDDSAVYYCARDSSNVGNAMDYWGQGTSVTVSS

SEQ ID NO: 645 - protein, 107 aa, Synthetic construct
DIQMTQTTSSLSASLGDRITISCRASQDISNYLNWYLQKPDGTIKLLIYYSSRLHSGVPSRFSGSGSGTDYSLTITNLEQEDIATYFCQQGHALPRTFGGGTKLEIK

SEQ ID NO: 646 - protein, 119 aa, Synthetic construct
EVQLQQSGPELVKPGASVKISCKGSGYTFTDYFMNWVKQSHGKSLEWVGDINPNNGDTTYSQKFMGKATLTVDKSSSTAYMELRSLTSEDSAVYHCAASGPPYVLLDYWGQGTSVTVSS

SEQ ID NO: 647 - protein, 107 aa, Synthetic construct
DIQMTQSPASLSASVGETVTITCRASENIYSYLAWYQQKQGKSPQLLVYNAKTLTEGVPTRFSGSGSGTQFSLKIDSLKPEDFGTYYCQHHYGTPLTFGAGTKLELN

SEQ ID NO: 648 - protein, 116 aa, Synthetic construct
QVQLQQSGTILARPGASVKMSCRASDYTFTDYWIQWIKQRPGQGLEWIGAIFPENGDTRYTQKFKGRATLTADKSSSTAYMQVNSLTSEDSAVYYCATFINYVDYWGQGTTLTVSS

SEQ ID NO: 649 - protein, 106 aa, Synthetic construct
QIVLIQSPAIMSASPGEKVTMTCSASSSVNNIHWYQQKSGTSPKRWIYDTTKLTSGVPARFSGSGSGTSYSLTISSMEAEDAATYYCQQWNINPYTFGGGTKLEIK

SEQ ID NO: 650 - protein, 119 aa, Synthetic construct
EVQLQQSGPELVKPGSLVKISCKTSGYTFTDYNMDWVKQSHGKSLEWIGAIDPKNGATSYNQKFKGKATLTVDKSSSTAYMELRSLTSEDSAVYYCARWDSNYWYFDVWGTGTTVTVSS

SEQ ID NO: 651 - protein, 107 aa, Synthetic construct
DIVMTQSQKIMSTSVGDRVSMTCKASQNIRSAVAWYQQKPGQSPKALIYLTSNRHTGVPDRFTGSGSGTDFTLAISDLQSEDLADYFCLQHWNYPYTFGGGTELEIK

SEQ ID NO: 652 - protein, 112 aa, Synthetic construct
EVQLVESGGGLVKPGGSLRLSCAASGFTFSDYYMYWVRQAPGKGLEWVSTISDAGGYTYYPDSVKGRFTISRDNAKNSLYLQMNSLRAEDTAVYYCAREDLWGQGTLVTVSS

SEQ ID NO: 653 - protein, 107 aa, Synthetic construct
DIQMTQSPSSLSASVGDRVTITCRASQDIGYSLNWFQQKPGKAPKRLIYATSRLDSGVPKRFSGSGSGTDFTLTISSLQPEDFATYYCLQYASFPYTFGGGTKLEIK

SEQ ID NO: 654 - protein, 112 aa, Synthetic construct
EVQLVESGGGLVKPGGSLRLSCAASGFTFSDYYMYWVRQAPGKGLEWVATISDAGGYTYYPDSVKGRFTISRDNAKNSLYLQMNSLRAEDTAVYYCGREDLWGQGTLVTVSS

SEQ ID NO: 655 - protein, 107 aa, Synthetic construct
DIQMTQSPSSLSASVGDRVTITCRASQDIGYSLNWFQQKPGKAPRRLIYATSRLDSGVPKRFSGSGSGTDFTLTISSLQPEDFATYYCLQYASFPYTFGGGTKLEIK

SEQ ID NO: 656 - protein, 112 aa, Synthetic construct
EVQLVESGGGLVKPGGSLRLSCAASGFTFSDYYMYWVRQAPGKGLEWVATISDAGGYTYYPDSVKGRFTISRDNAKNSLYLQMNSLRAEDTAVYFCGREDLWGQGTLVTVSS

SEQ ID NO: 657 - protein, 447 aa, synthetic construct
QVQLVQSGAEVKKPGASVKVSCKASGYTFTDYNINWVRQAPGQGLEWMGYIYPYIGGSGYAQKFQGRVTMTRDTSTSTVYMELSSLRSEDTAVYYCAREDKTARNAMDYWGQGTLVTVSSASTKGPSVFPLAPCSRSTSESTAALGCLVKDYFPEPVTVSWNSGALTSGVHTFPAVLQSSGLYSLSSVVTVPSSSLGTKTYTCNVDHKPSNTKVDKRVESKYGPPCPPCPAPEFLGGPSVFLFPPKPKDTLMISRTPEVTCVVVDVSQEDPEVQFNWYVDGVEVHNAKTKPREEQFNSTYRVVSVLTVLHQDWLNGKEYKCKVSNKGLPSSIEKTISKAKGQPREPQVYTLPPSQEEMTKNQVSLTCLVKGFYPSDIAVEWESNGQPENNYKTTPPVLDSDGSFFLYSRLTVDKSRWQEGNVFSCSVMHEALHNHYTQKSLSLSPGK

SEQ ID NO: 658 - protein, 214 aa, synthetic construct
DIQMTQSPSSLSASVGDRVTITCRVSENIYSNLAWYQQKPGKAPKLLIYEATNLAEGVPSRFSGSGSGTDFTLTISSLQPEDFATYYCQHFWGTPYTFGQGTKLEIKRTVAAPSVFIFPPSDEQLKSGTASVVCLLNNFYPREAKVQWKVDNALQSGNSQESVTEQDSKDSTYSLSSTLTLSKADYEKHKVYACEVTHQGLSSPVTKSFNRGEC

SEQ ID NO: 659 - protein, 330 aa, synthetic construct [sequence omitted]

SEQ ID NO: 660 - protein, 107 aa, synthetic construct [sequence omitted]

SEQ ID NO: 661 - protein, 232 aa, synthetic construct
EPKSCDKTHTCPPCPAPELLGGPSVFLFPPKPKDTLMISRTPEVTCVVVDVSHEDPEVKFNWYVDGVEVHNAKTKPREEQYNSTYRVVSVLTVLHQDWLNGKEYKCKVSNKALPAPIEKTISKAKGQPREPQVYTLPPSRDELTKNQVSLTCLVKGFYPSDIAVEWESNGQPENNYKTTPPVLDSDGSFFLYSKLTVDKSRWQQGNVFSCSVMHEALHNHYTQKSLSLSPGK

SEQ ID NO: 662 - DNA, 978 bp, synthetic construct
  source 1..978: mol_type = other DNA
atgagaacagaggcccaagtgcctgctctgcagcctccggagcctggcctggaaggcgccatgggccaccggaccctggtgctgccttgggtcctgctgaccctgtgtgtgaccgccggcacacctgaggtgtgggtgcaggttagaatggaggccacagagctgagctcttttaccatccggtgcggattcctgggatccggcagcatttctctggtcaccgtgtcttggggcggacctaatggcgctggcggcaccacactggccgtgctgcaccctgagcggggcatcagacagtgggcccctgccagacaggccagatgggaaacccagagcagcatctctctgatcctggaaggaagcggcgccagcagcccctgcgccaacacaacattctgctgcaagttcgcctccttcccagagggaagctgggaggcctgcggcagcctgcctcctagcagtgatcccggcctcagcgcccctcctacccctgctccaatcctgagagccgacctggccggaatcctgggcgtgtccggcgtgctgcttttcggctgcgtgtacctgctgcatctgctgaggcggcacaagcacagaccagcccctagactgcaaccttctagaaccagccctcaggcccctcgcgcccgggcttgggcccctagccaggcctctcaggctgctctgcatgtgccctacgcaaccatcaacaccagctgtagacctgccaccctggacaccgcccacccccacggaggcccaagctggtgggccagcctgcccacccacgccgcccacagaccccagggccccgccgcttgggctagcacccctatccccgcaagaggcagctttgtgtccgtggaaaacggcctgtacgcccaggccggcgagagacctccacacacaggccctggcctgacactgttccccgacccccggggccccagagccatggaaggccctctgggcgtgcgg